European Patent Application EP 4 772 622 A2, published July 8, 2026. Title: CRISPR ENZYMES AND SYSTEMS WITH MODIFIED PAM SPECIFICITY. Applicant: THE BROAD INSTITUTE, INC. Application US 19/262,704, filed July 8, 2025. The sequence listing filed with the application follows.

SEQUENCE LISTING (482 sequences)

SEQ ID NO: 1 - protein, 7 aa, Simian virus 40
PKKKRKV

SEQ ID NO: 2 - protein, 16 aa, unidentified
  REGION 1..16: note = Description of Unknown: Nucleoplasmin bipartite NLS sequence
KRPAATKKAGQAKKKK

SEQ ID NO: 3 - protein, 9 aa, unidentified
  REGION 1..9: note = Description of Unknown: C-myc NLS sequence
PAAKRVKLD

SEQ ID NO: 4 - protein, 11 aa, unidentified
  REGION 1..11: note = Description of Unknown: C-myc NLS sequence
RQRRNELKRSP

SEQ ID NO: 5 - protein, 38 aa, Homo sapiens
NQSSNFGPMKGGNFGGRSSGPYGGGGQYFAKPRNQGGY

SEQ ID NO: 6 - protein, 42 aa, unidentified
  REGION 1..42: note = Description of Unknown: IBB domain from importin-alpha sequence
RMRIZFKNKGKDTAELRRRRVEVSVELRKAKKDEQILKRRNV

SEQ ID NO: 7 - protein, 8 aa, unidentified
  REGION 1..8: note = Description of Unknown: Myoma T protein sequence
VSRKRPRP

SEQ ID NO: 8 - protein, 8 aa, unidentified
  REGION 1..8: note = Description of Unknown: Myoma T protein sequence
PPKKARED

SEQ ID NO: 9 - protein, 8 aa, Homo sapiens
PQPKKKPL

SEQ ID NO: 10 - protein, 12 aa, Mus musculus
SALIKKKKKMAP

SEQ ID NO: 11 - protein, 5 aa, Influenza virus
DRLRR

SEQ ID NO: 12 - protein, 7 aa, Influenza virus
PKQKKRK

SEQ ID NO: 13 - protein, 10 aa, Hepatitis delta virus
RKLKKKIKKL

SEQ ID NO: 14 - protein, 10 aa, Mus musculus
REKKKFLKRR

SEQ ID NO: 15 - protein, 20 aa, Homo sapiens
KRKGDEVDGVDEVAKKKSKK

SEQ ID NO: 16 - protein, 17 aa, Homo sapiens
RKCLQAGMNLEARKTKK

SEQ ID NO: 17 - protein, 4 aa, synthetic construct
  REGION 1..4: note = Description of Artificial Sequence: Synthetic peptide
GGGS

SEQ ID NO: 18 - protein, 15 aa, synthetic construct
  REGION 1..15: note = Description of Artificial Sequence: Synthetic peptide
GGGGSGGGGSGGGGS

SEQ ID NO: 19 - protein, 30 aa, synthetic construct
  REGION 1..30: note = Description of Artificial Sequence: Synthetic polypeptide
GGGGSGGGGSGGGGSGGGGSGGGGSGGGGS

SEQ ID NO: 20 - protein, 45 aa, synthetic construct
  REGION 1..45: note = Description of Artificial Sequence: Synthetic polypeptide
GGGGSGGGGSGGGGSGGGGSGGGGSGGGGSGGGGSGGGGSGGGGS

SEQ ID NO: 21 - protein, 60 aa, synthetic construct
  REGION 1..60: note = Description of Artificial Sequence: Synthetic polypeptide
GGGGSGGGGSGGGGSGGGGSGGGGSGGGGSGGGGSGGGGSGGGGSGGGGSGGGGSGGGGS

SEQ ID NO: 22 - protein, 5 aa, synthetic construct
  REGION 1..5: note = Description of Artificial Sequence: Synthetic peptide
GGGGS

SEQ ID NO: 23 - protein, 10 aa, synthetic construct
  REGION 1..10: note = Description of Artificial Sequence: Synthetic peptide
GGGGSGGGGS

SEQ ID NO: 24 - protein, 20 aa, synthetic construct
  REGION 1..20: note = Description of Artificial Sequence: Synthetic peptide
GGGGSGGGGSGGGGSGGGGS

SEQ ID NO: 25 - protein, 25 aa, synthetic construct
  REGION 1..25: note = Description of Artificial Sequence: Synthetic peptide
GGGGSGGGGSGGGGSGGGGSGGGGS

SEQ ID NO: 26 - protein, 35 aa, synthetic construct
  REGION 1..35: note = Description of Artificial Sequence: Synthetic polypeptide
GGGGSGGGGSGGGGSGGGGSGGGGSGGGGSGGGGS

SEQ ID NO: 27 - protein, 40 aa, synthetic construct
  REGION 1..40: note = Description of Artificial Sequence: Synthetic polypeptide
GGGGSGGGGSGGGGSGGGGSGGGGSGGGGSGGGGSGGGGS

SEQ ID NO: 28 - protein, 50 aa, synthetic construct
  REGION 1..50: note = Description of Artificial Sequence: Synthetic polypeptide
GGGGSGGGGSGGGGSGGGGSGGGGSGGGGSGGGGSGGGGSGGGGSGGGGS

SEQ ID NO: 29 - protein, 55 aa, synthetic construct
  REGION 1..55: note = Description of Artificial Sequence: Synthetic polypeptide
GGGGSGGGGSGGGGSGGGGSGGGGSGGGGSGGGGSGGGGSGGGGSGGGGSGGGGS

SEQ ID NO: 30 - RNA, 120 nt, synthetic construct
  misc_feature 1..120: note = Description of Artificial Sequence: Synthetic polynucleotide
  misc_feature 1..120: note = See specification as filed for detailed description of substitutions and preferred embodiments
  source 1..120: mol_type = other RNA
aaaaaaaaaaaaaaaaaaaaaaaaaaaaaaaaaaaaaaaaaaaaaaaaaaaaaaaaaaaaaaaaaaaaaaaaaaaaaaaaaaaaaaaaaaaaaaaaaaaaaaaaaaaaaaaaaaaaaaaa

SEQ ID NO: 31 - protein, 12 aa, synthetic construct
  REGION 1..12: note = Description of Artificial Sequence: Synthetic peptide
  SITE 2: note = 6-aminohexanoic acid
  SITE 5: note = 6-aminohexanoic acid
  SITE 8: note = 6-aminohexanoic acid
  SITE 11: note = 6-aminohexanoic acid
RXRRXRRXRRXR

SEQ ID NO: 32 - DNA, 20 bp, synthetic construct
  misc_feature 1..20: note = Description of Artificial Sequence: Synthetic oligonucleotide
  source 1..20: mol_type = other DNA
ctgaattagctgtatcgtca

SEQ ID NO: 33 - DNA, 20 bp, synthetic construct
  misc_feature 1..20: note = Description of Artificial Sequence: Synthetic oligonucleotide
  source 1..20: mol_type = other DNA
gaatataaacttgtggtagt

SEQ ID NO: 34 - DNA, 20 bp, Homo sapiens
  source 1..20: mol_type = unassigned DNA
gagtccgagcagaagaagaa

SEQ ID NO: 35 - DNA, 20 bp, Homo sapiens
  source 1..20: mol_type = unassigned DNA
gagtcctagcaggagaagaa

SEQ ID NO: 36 - DNA, 20 bp, Homo sapiens
  source 1..20: mol_type = unassigned DNA
gagtctaagcagaagaagaa

SEQ ID NO: 37 - protein, 4 aa, synthetic construct
  REGION 1..4: note = Description of Artificial Sequence: Synthetic peptide
GGSG

SEQ ID NO: 38 - protein, 7 aa, synthetic construct
  REGION 1..7: note = Description of Artificial Sequence: Synthetic peptide
AEAAAKA

SEQ ID NO: 39 - protein, 9 aa, unidentified
  REGION 1..9: note = Description of Unknown: "LAGLIDADG" family peptide motif sequence
LAGLIDADG

SEQ ID NO: 40 - DNA, 42 bp, synthetic construct
  misc_feature 1..42: note = Description of Artificial Sequence: Synthetic oligonucleotide
  source 1..42: mol_type = other DNA
acactggcccggggctgggacgtgaataaggagaagaacaat

SEQ ID NO: 41 - DNA, 42 bp, synthetic construct
  misc_feature 1..42: note = Description of Artificial Sequence: Synthetic oligonucleotide
  source 1..42: mol_type = other DNA
acactggcctcaggctgggacgtgaagaaggagaagaacaat

SEQ ID NO: 42 - DNA, 42 bp, synthetic construct
  misc_feature 1..42: note = Description of Artificial Sequence: Synthetic oligonucleotide
  source 1..42: mol_type = other DNA
acactggcctcaggctgggacgtgaatgccgagaagaacaat

SEQ ID NO: 43 - DNA, 42 bp, synthetic construct
  misc_feature 1..42: note = Description of Artificial Sequence: Synthetic oligonucleotide
  source 1..42: mol_type = other DNA
acactggcctcaggctgggacgtgaatcacgagaagaacaat

SEQ ID NO: 44 - DNA, 42 bp, synthetic construct
  misc_feature 1..42: note = Description of Artificial Sequence: Synthetic oligonucleotide
  source 1..42: mol_type = other DNA
acactggcctcaggctgggacgtgaataacgagaagaacaat

SEQ ID NO: 45 - DNA, 42 bp, synthetic construct
  misc_feature 1..42: note = Description of Artificial Sequence: Synthetic oligonucleotide
  source 1..42: mol_type = other DNA
acactggcctcaggctgggacgtgaatcaggagaagaacaat

SEQ ID NO: 46 - DNA, 42 bp, synthetic construct
  misc_feature 1..42: note = Description of Artificial Sequence: Synthetic oligonucleotide
  source 1..42: mol_type = other DNA
acactggcctcaggctgggacgtgaatcgggagaagaacaat

SEQ ID NO: 47 - DNA, 42 bp, synthetic construct
  misc_feature 1..42: note = Description of Artificial Sequence: Synthetic oligonucleotide
  source 1..42: mol_type = other DNA
acactggcctcaggctgggacgtgaataaggagtacaacaat

SEQ ID NO: 48 - DNA, 42 bp, synthetic construct
  misc_feature 1..42: note = Description of Artificial Sequence: Synthetic oligonucleotide
  source 1..42: mol_type = other DNA
acactggcctcaggctgggacgtgaataaggagaagcggaat

SEQ ID NO: 49 - DNA, 42 bp, synthetic construct
  misc_feature 1..42: note = Description of Artificial Sequence: Synthetic oligonucleotide
  source 1..42: mol_type = other DNA
acactggcctcaggctgggacgtgaataaggagaagaacggc

SEQ ID NO: 50 - DNA, 42 bp, synthetic construct
  misc_feature 1..42: note = Description of Artificial Sequence: Synthetic oligonucleotide
  source 1..42: mol_type = other DNA
acactggcctcaggctgggacgtgaataaggagaagaacaag

SEQ ID NO: 51 - DNA, 42 bp, synthetic construct
  misc_feature 1..42: note = Description of Artificial Sequence: Synthetic oligonucleotide
  source 1..42: mol_type = other DNA
acactggcctcaggctgggacgtgaataaggagaagaaccgg

SEQ ID NO: 52 - DNA, 42 bp, synthetic construct
  misc_feature 1..42: note = Description of Artificial Sequence: Synthetic oligonucleotide
  source 1..42: mol_type = other DNA
acactggcctcaggctgggacgtgaataaggagaagaacagc

SEQ ID NO: 53 - DNA, 42 bp, synthetic construct
  misc_feature 1..42: note = Description of Artificial Sequence: Synthetic oligonucleotide
  source 1..42: mol_type = other DNA
acactggcctcaggctgggacgtgaataaggagaagaacacc

SEQ ID NO: 54 - DNA, 44 bp, synthetic construct
  misc_feature 1..44: note = Description of Artificial Sequence: Synthetic oligonucleotide
  source 1..44: mol_type = other DNA
atgccgccaagatgatcccagcctgcagcacccagctgaaggcg

SEQ ID NO: 55 - DNA, 44 bp, synthetic construct
  misc_feature 1..44: note = Description of Artificial Sequence: Synthetic oligonucleotide
  source 1..44: mol_type = other DNA
atgccgccaagatgatcccacggtgcagcacccagctgaaggcg

SEQ ID NO: 56 - DNA, 42 bp, synthetic construct
  misc_feature 1..42: note = Description of Artificial Sequence: Synthetic oligonucleotide
  source 1..42: mol_type = other DNA
acactggcccggggctgggacgtgaatcgggagaagaacaat

SEQ ID NO: 57 - DNA, 42 bp, synthetic construct
  misc_feature 1..42: note = Description of Artificial Sequence: Synthetic oligonucleotide
  source 1..42: mol_type = other DNA
acactggcctcaggctgggacgtgaatcgggagaagaaccgg

SEQ ID NO: 58 - DNA, 42 bp, synthetic construct
  misc_feature 1..42: note = Description of Artificial Sequence: Synthetic oligonucleotide
  source 1..42: mol_type = other DNA
acactggcccggggctgggacgtgaataaggagtacaacaat

SEQ ID NO: 59 - DNA, 42 bp, synthetic construct
  misc_feature 1..42: note = Description of Artificial Sequence: Synthetic oligonucleotide
  source 1..42: mol_type = other DNA
acactggcccggggctgggacgtgaatcgggagtacaacaat

SEQ ID NO: 60 - DNA, 42 bp, synthetic construct
  misc_feature 1..42: note = Description of Artificial Sequence: Synthetic oligonucleotide
  source 1..42: mol_type = other DNA
cggctggcctcaggctgggacgtgaataaggagaagaacaat

SEQ ID NO: 61 - DNA, 42 bp, synthetic construct
  misc_feature 1..42: note = Description of Artificial Sequence: Synthetic oligonucleotide
  source 1..42: mol_type = other DNA
aagctggcctcaggctgggacgtgaataaggagaagaacaat

SEQ ID NO: 62 - DNA, 42 bp, synthetic construct
  misc_feature 1..42: note = Description of Artificial Sequence: Synthetic oligonucleotide
  source 1..42: mol_type = other DNA
acactggcctcaggctgggacgtgaatggcgagaagaacaat

SEQ ID NO: 63 - DNA, 42 bp, synthetic construct
  misc_feature 1..42: note = Description of Artificial Sequence: Synthetic oligonucleotide
  source 1..42: mol_type = other DNA
acactggcctcaggctgggacgtgaattgcgagaagaacaat

SEQ ID NO: 64 - DNA, 42 bp, synthetic construct
  misc_feature 1..42: note = Description of Artificial Sequence: Synthetic oligonucleotide
  source 1..42: mol_type = other DNA
acactggcctcaggctgggacgtgaatttcgagaagaacaat

SEQ ID NO: 65 - DNA, 42 bp, synthetic construct
  misc_feature 1..42: note = Description of Artificial Sequence: Synthetic oligonucleotide
  source 1..42: mol_type = other DNA
acactggcctcaggctgggacgtgaatatcgagaagaacaat

SEQ ID NO: 66 - DNA, 42 bp, synthetic construct
  misc_feature 1..42: note = Description of Artificial Sequence: Synthetic oligonucleotide
  source 1..42: mol_type = other DNA
acactggcctcaggctgggacgtgaatatggagaagaacaat

SEQ ID NO: 67 - DNA, 42 bp, synthetic construct
  misc_feature 1..42: note = Description of Artificial Sequence: Synthetic oligonucleotide
  source 1..42: mol_type = other DNA
acactggcctcaggctgggacgtgaatagcgagaagaacaat

SEQ ID NO: 68 - DNA, 42 bp, synthetic construct
  misc_feature 1..42: note = Description of Artificial Sequence: Synthetic oligonucleotide
  source 1..42: mol_type = other DNA
acactggcctcaggctgggacgtgaataccgagaagaacaat

SEQ ID NO: 69 - DNA, 42 bp, synthetic construct
  misc_feature 1..42: note = Description of Artificial Sequence: Synthetic oligonucleotide
  source 1..42: mol_type = other DNA
acactggcctcaggctgggacgtgaatgtggagaagaacaat

SEQ ID NO: 70 - DNA, 42 bp, synthetic construct
  misc_feature 1..42: note = Description of Artificial Sequence: Synthetic oligonucleotide
  source 1..42: mol_type = other DNA
acactggcctcaggctgggacgtgaattgggagaagaacaat

SEQ ID NO: 71 - DNA, 42 bp, synthetic construct
  misc_feature 1..42: note = Description of Artificial Sequence: Synthetic oligonucleotide
  source 1..42: mol_type = other DNA
acactggcctcaggctgggacgtgaattacgagaagaacaat

SEQ ID NO: 72 - DNA, 42 bp, synthetic construct
  misc_feature 1..42: note = Description of Artificial Sequence: Synthetic oligonucleotide
  source 1..42: mol_type = other DNA
acactggcctcaggctgggacgtgaatgacgagaagaacaat

SEQ ID NO: 73 - DNA, 42 bp, synthetic construct
  misc_feature 1..42: note = Description of Artificial Sequence: Synthetic oligonucleotide
  source 1..42: mol_type = other DNA
acactggcctcaggctgggacgtgaatgaggagaagaacaat

SEQ ID NO: 74 - DNA, 42 bp, synthetic construct
  misc_feature 1..42: note = Description of Artificial Sequence: Synthetic oligonucleotide
  source 1..42: mol_type = other DNA
acactggcctcaggctgggacgtgaatctggagaagaacaat

SEQ ID NO: 75 - DNA, 42 bp, synthetic construct
  misc_feature 1..42: note = Description of Artificial Sequence: Synthetic oligonucleotide
  source 1..42: mol_type = other DNA
acactggcctcaggctgggacgtgaatcccgagaagaacaat

SEQ ID NO: 76 - DNA, 42 bp, synthetic construct
  misc_feature 1..42: note = Description of Artificial Sequence: Synthetic oligonucleotide
  source 1..42: mol_type = other DNA
acactggcccggggctgggacgtgaatgtggagaagaacaat

SEQ ID NO: 77 - DNA, 42 bp, synthetic construct
  misc_feature 1..42: note = Description of Artificial Sequence: Synthetic oligonucleotide
  source 1..42: mol_type = other DNA
acactggcctcaggctgggacgtgaatgtggagaagaaccgg

SEQ ID NO: 78 - DNA, 42 bp, synthetic construct
  misc_feature 1..42: note = Description of Artificial Sequence: Synthetic oligonucleotide
  source 1..42: mol_type = other DNA
acactggcccggggctgggacgtgaatgtggagaagaaccgg

SEQ ID NO: 79 - DNA, 42 bp, synthetic construct
  misc_feature 1..42: note = Description of Artificial Sequence: Synthetic oligonucleotide
  source 1..42: mol_type = other DNA
acactggcccggggctgggacgtgaatgtggagaagcggcgg

SEQ ID NO: 80 - DNA, 42 bp, synthetic construct
  misc_feature 1..42: note = Description of Artificial Sequence: Synthetic oligonucleotide
  source 1..42: mol_type = other DNA
acactggcccggggctgggacgtgaagaaggagaagaacaat

SEQ ID NO: 81 - DNA, 42 bp, synthetic construct
  misc_feature 1..42: note = Description of Artificial Sequence: Synthetic oligonucleotide
  source 1..42: mol_type = other DNA
acactggcccggggctgggacgtgaataaggagaagcggaat

SEQ ID NO: 82 - DNA, 42 bp, synthetic construct
  misc_feature 1..42: note = Description of Artificial Sequence: Synthetic oligonucleotide
  source 1..42: mol_type = other DNA
acactggcccggggctgggacgtgaataaggagaagaacagc

SEQ ID NO: 83 - DNA, 42 bp, synthetic construct
  misc_feature 1..42: note = Description of Artificial Sequence: Synthetic oligonucleotide
  source 1..42: mol_type = other DNA
acactggcccggggctgggacgtgaagaaggagtacaacaat

SEQ ID NO: 84 - DNA, 42 bp, synthetic construct
  misc_feature 1..42: note = Description of Artificial Sequence: Synthetic oligonucleotide
  source 1..42: mol_type = other DNA
acactggcccggggctgggacgtgaagaaggagaagcggaat

SEQ ID NO: 85 - DNA, 42 bp, synthetic construct
  misc_feature 1..42: note = Description of Artificial Sequence: Synthetic oligonucleotide
  source 1..42: mol_type = other DNA
acactggcccggggctgggacgtgaagaaggagaagaacagc

SEQ ID NO: 86 - DNA, 42 bp, synthetic construct
  misc_feature 1..42: note = Description of Artificial Sequence: Synthetic oligonucleotide
  source 1..42: mol_type = other DNA
acactggcccggggctgggacgtgaataaggagtaccggaat

SEQ ID NO: 87 - DNA, 42 bp, synthetic construct
  misc_feature 1..42: note = Description of Artificial Sequence: Synthetic oligonucleotide
  source 1..42: mol_type = other DNA
acactggcccggggctgggacgtgaataaggagtacaacagc

SEQ ID NO: 88 - DNA, 42 bp, synthetic construct
  misc_feature 1..42: note = Description of Artificial Sequence: Synthetic oligonucleotide
  source 1..42: mol_type = other DNA
acactggcccggggctgggacgtgaataaggagaagcggagc

SEQ ID NO: 89 - DNA, 42 bp, synthetic construct
  misc_feature 1..42: note = Description of Artificial Sequence: Synthetic oligonucleotide
  source 1..42: mol_type = other DNA
acactggcccggggctgggacgtgaagaaggagtaccggagc

SEQ ID NO: 90 - DNA, 42 bp, synthetic construct
  misc_feature 1..42: note = Description of Artificial Sequence: Synthetic oligonucleotide
  source 1..42: mol_type = other DNA
acactggcctcaggctgggacgtgaatgtggagaagaacggc

SEQ ID NO: 91 - DNA, 42 bp, synthetic construct
  misc_feature 1..42: note = Description of Artificial Sequence: Synthetic oligonucleotide
  source 1..42: mol_type = other DNA
acactggcccggggctgggacgtgaatgtggagaagaacggc

SEQ ID NO: 92 - DNA, 42 bp, synthetic construct
  misc_feature 1..42: note = Description of Artificial Sequence: Synthetic oligonucleotide
  source 1..42: mol_type = other DNA
acactggcccggggctgggacgtgaatgtggagaagcggggc

SEQ ID NO: 93 - DNA, 23 bp, unidentified
  misc_feature 1..23: note = Description of Unknown: Target sequence
  source 1..23: mol_type = unassigned DNA
aaggaggaggaagctgctaagga

SEQ ID NO: 94 - DNA, 23 bp, unidentified
  misc_feature 1..23: note = Description of Unknown: Target sequence
  source 1..23: mol_type = unassigned DNA
actagggtgggcaaccacaaacc

SEQ ID NO: 95 - DNA, 23 bp, unidentified
  misc_feature 1..23: note = Description of Unknown: Target sequence
  source 1..23: mol_type = unassigned DNA
cctctttagccagagccggggtg

SEQ ID NO: 96 - DNA, 23 bp, unidentified
  misc_feature 1..23: note = Description of Unknown: Target sequence
  source 1..23: mol_type = unassigned DNA
agggcgttggagcggggagaagg

SEQ ID NO: 97 - DNA, 23 bp, unidentified
  misc_feature 1..23: note = Description of Unknown: Target sequence
  source 1..23: mol_type = unassigned DNA
gagcggggagaaggccaggggtc

SEQ ID NO: 98 - DNA, 23 bp, unidentified
  misc_feature 1..23: note = Description of Unknown: Target sequence
  source 1..23: mol_type = unassigned DNA
aaattccagcaccgagcgccctg

SEQ ID NO: 99 - DNA, 23 bp, unidentified
  misc_feature 1..23: note = Description of Unknown: Target sequence
  source 1..23: mol_type = unassigned DNA
tagctgtttgggaggtcagaaat

SEQ ID NO: 100 - DNA, 23 bp, unidentified
  misc_feature 1..23: note = Description of Unknown: Target sequence
  source 1..23: mol_type = unassigned DNA
tctttagccagagccggggtgtg

SEQ ID NO: 101 - DNA, 23 bp, unidentified
  misc_feature 1..23: note = Description of Unknown: Target sequence
  source 1..23: mol_type = unassigned DNA
cgctccaacgccctcaaccccac

SEQ ID NO: 102 - DNA, 23 bp, unidentified
  misc_feature 1..23: note = Description of Unknown: Target sequence
  source 1..23: mol_type = unassigned DNA
tggccaggctttggggaggcctg

SEQ ID NO: 103 - DNA, 23 bp, unidentified
  misc_feature 1..23: note = Description of Unknown: Target sequence
  source 1..23: mol_type = unassigned DNA
tctgtcaatggcggccccgggct

SEQ ID NO: 104 - DNA, 23 bp, unidentified
  misc_feature 1..23: note = Description of Unknown: Target sequence
  source 1..23: mol_type = unassigned DNA
gtcacccctgtttctggcaccag

SEQ ID NO: 105 - DNA, 23 bp, unidentified
  misc_feature 1..23: note = Description of Unknown: Target sequence
  source 1..23: mol_type = unassigned DNA
cccgctccaacgccctcaacccc

SEQ ID NO: 106 - DNA, 23 bp, unidentified
  misc_feature 1..23: note = Description of Unknown: Target sequence
  source 1..23: mol_type = unassigned DNA
gctaaagagggaatgggctttgg

SEQ ID NO: 107 - DNA, 23 bp, unidentified
  misc_feature 1..23: note = Description of Unknown: Target sequence
  source 1..23: mol_type = unassigned DNA
tgtgggtgagtgagtgtgtgcgt

SEQ ID NO: 108 - DNA, 23 bp, unidentified
  misc_feature 1..23: note = Description of Unknown: Target sequence
  source 1..23: mol_type = unassigned DNA
ccctcccgtcacccctgtttctg

SEQ ID NO: 109 - DNA, 23 bp, unidentified
  misc_feature 1..23: note = Description of Unknown: Target sequence
  source 1..23: mol_type = unassigned DNA
aatggcggccccgggcttcaagc

SEQ ID NO: 110 - DNA, 23 bp, unidentified
  misc_feature 1..23: note = Description of Unknown: Target sequence
  source 1..23: mol_type = unassigned DNA
ggtgagtgagtgtgtgcgtgtgg

SEQ ID NO: 111 - DNA, 23 bp, unidentified
  misc_feature 1..23: note = Description of Unknown: Target sequence
  source 1..23: mol_type = unassigned DNA
aaagcccattccctctttagcca

SEQ ID NO: 112 - DNA, 23 bp, unidentified
  misc_feature 1..23: note = Description of Unknown: Target sequence
  source 1..23: mol_type = unassigned DNA
ctctttagccagagccggggtgt

SEQ ID NO: 113 - DNA, 23 bp, unidentified
  misc_feature 1..23: note = Description of Unknown: Target sequence
  source 1..23: mol_type = unassigned DNA
tggtgccagaaacaggggtgacg

SEQ ID NO: 114 - DNA, 23 bp, unidentified
  misc_feature 1..23: note = Description of Unknown: Target sequence
  source 1..23: mol_type = unassigned DNA
ctgatggtccatgtctgttactc

SEQ ID NO: 115 - DNA, 23 bp, unidentified
  misc_feature 1..23: note = Description of Unknown: Target sequence
  source 1..23: mol_type = unassigned DNA
gctgaagggaaataaaaggaaaa

SEQ ID NO: 116 - DNA, 23 bp, unidentified
  misc_feature 1..23: note = Description of Unknown: Target sequence
  source 1..23: mol_type = unassigned DNA
gccaccacagggaagctgggtga

SEQ ID NO: 117 - DNA, 23 bp, unidentified
  misc_feature 1..23: note = Description of Unknown: Target sequence
  source 1..23: mol_type = unassigned DNA
aattccagcaccgagcgccctgg

SEQ ID NO: 118 - DNA, 23 bp, unidentified
  misc_feature 1..23: note = Description of Unknown: Target sequence
  source 1..23: mol_type = unassigned DNA
aaaattttacaccacaaaatgtt

SEQ ID NO: 119 - DNA, 23 bp, unidentified
  misc_feature 1..23: note = Description of Unknown: Target sequence
  source 1..23: mol_type = unassigned DNA
tatttctgacctcccaaacagct

SEQ ID NO: 120 - DNA, 23 bp, unidentified
  misc_feature 1..23: note = Description of Unknown: Target sequence
  source 1..23: mol_type = unassigned DNA
atgaatatcaaattccagcaccg

SEQ ID NO: 121 - DNA, 23 bp, unidentified
  misc_feature 1..23: note = Description of Unknown: Target sequence
  source 1..23: mol_type = unassigned DNA
catcaaccggtggcgcattgcca

SEQ ID NO: 122 - DNA, 23 bp, unidentified
  misc_feature 1..23: note = Description of Unknown: Target sequence
  source 1..23: mol_type = unassigned DNA
gagccggggtgtgcagacggcag

SEQ ID NO: 123 - DNA, 23 bp, unidentified
  misc_feature 1..23: note = Description of Unknown: Target sequence
  source 1..23: mol_type = unassigned DNA
ttaaagaaaatatcatctttggt

SEQ ID NO: 124 - DNA, 23 bp, unidentified
  misc_feature 1..23: note = Description of Unknown: Target sequence
  source 1..23: mol_type = unassigned DNA
agcgccccctagtgactgccgtc

SEQ ID NO: 125 - DNA, 23 bp, unidentified
  misc_feature 1..23: note = Description of Unknown: Target sequence
  source 1..23: mol_type = unassigned DNA
tccccattggcctgcttcgtggc

SEQ ID NO: 126 - DNA, 23 bp, unidentified
  misc_feature 1..23: note = Description of Unknown: Target sequence
  source 1..23: mol_type = unassigned DNA
gtcagcggactcaccggccaggg

SEQ ID NO: 127 - DNA, 23 bp, unidentified
  misc_feature 1..23: note = Description of Unknown: Target sequence
  source 1..23: mol_type = unassigned DNA
ttccctctttagccagagccggg

SEQ ID NO: 128 - DNA, 23 bp, unidentified
  misc_feature 1..23: note = Description of Unknown: Target sequence
  source 1..23: mol_type = unassigned DNA
ggcttcaagccctgtggggccat

SEQ ID NO: 129 - DNA, 23 bp, unidentified
  misc_feature 1..23: note = Description of Unknown: Target sequence
  source 1..23: mol_type = unassigned DNA
aagatgatattttctttaatggt

SEQ ID NO: 130 - DNA, 23 bp, unidentified
  misc_feature 1..23: note = Description of Unknown: Target sequence
  source 1..23: mol_type = unassigned DNA
ctgtggtggccgagcgcccccta

SEQ ID NO: 131 - DNA, 23 bp, unidentified
  misc_feature 1..23: note = Description of Unknown: Target sequence
  source 1..23: mol_type = unassigned DNA
tctgcacaccccggctctggcta

SEQ ID NO: 132 - DNA, 23 bp, unidentified
  misc_feature 1..23: note = Description of Unknown: Target sequence
  source 1..23: mol_type = unassigned DNA
atgtcctccccattggcctgctt

SEQ ID NO: 133 - DNA, 23 bp, unidentified
  misc_feature 1..23: note = Description of Unknown: Target sequence
  source 1..23: mol_type = unassigned DNA
caaatatgtagctgtttgggagg

SEQ ID NO: 134 - DNA, 23 bp, unidentified
  misc_feature 1..23: note = Description of Unknown: Target sequence
  source 1..23: mol_type = unassigned DNA
ctccattcacccagcttccctgt

SEQ ID NO: 135 - DNA, 23 bp, unidentified
  misc_feature 1..23: note = Description of Unknown: Target sequence
  source 1..23: mol_type = unassigned DNA
aggaaaactgagaacagaatgaa

SEQ ID NO: 136 - DNA, 23 bp, unidentified
  misc_feature 1..23: note = Description of Unknown: Target sequence
  source 1..23: mol_type = unassigned DNA
taaactcattaatgcccttcggc

SEQ ID NO: 137 - DNA, 23 bp, unidentified
  misc_feature 1..23: note = Description of Unknown: Target sequence
  source 1..23: mol_type = unassigned DNA
atgtcacctccaatgactagggt

SEQ ID NO: 138 - DNA, 23 bp, unidentified
  misc_feature 1..23: note = Description of Unknown: Target sequence
  source 1..23: mol_type = unassigned DNA
tggcaatgcgccaccggttgatg

SEQ ID NO: 139 - DNA, 23 bp, unidentified
  misc_feature 1..23: note = Description of Unknown: Target sequence
  source 1..23: mol_type = unassigned DNA
gcgatgttttttctggagattta

SEQ ID NO: 140 - DNA, 23 bp, unidentified
  misc_feature 1..23: note = Description of Unknown: Target sequence
  source 1..23: mol_type = unassigned DNA
cagggaagctgggtgaatggagc

SEQ ID NO: 141 - DNA, 23 bp, unidentified
  misc_feature 1..23: note = Description of Unknown: Target sequence
  source 1..23: mol_type = unassigned DNA
ccacagggaagctgggtgaatgg

SEQ ID NO: 142 - DNA, 23 bp, unidentified
  misc_feature 1..23: note = Description of Unknown: Target sequence
  source 1..23: mol_type = unassigned DNA
gggtgtgcagacggcagtcacta

SEQ ID NO: 143 - DNA, 23 bp, unidentified
  misc_feature 1..23: note = Description of Unknown: Target sequence
  source 1..23: mol_type = unassigned DNA
tgggctctctgtacatgaagcaa

SEQ ID NO: 144 - DNA, 23 bp, unidentified
  misc_feature 1..23: note = Description of Unknown: Target sequence
  source 1..23: mol_type = unassigned DNA
gaaatagggggtccaggagcaaa

SEQ ID NO: 145 - DNA, 23 bp, unidentified
  misc_feature 1..23: note = Description of Unknown: Target sequence
  source 1..23: mol_type = unassigned DNA
cctagtgactgccgtctgcacac

SEQ ID NO: 146 - DNA, 23 bp, unidentified
  misc_feature 1..23: note = Description of Unknown: Target sequence
  source 1..23: mol_type = unassigned DNA
gccagggcgctcggtgctggaat

SEQ ID NO: 147 - DNA, 23 bp, unidentified
  misc_feature 1..23: note = Description of Unknown: Target sequence
  source 1..23: mol_type = unassigned DNA
attccctctttagccagagccgg

SEQ ID NO: 148 - DNA, 23 bp, unidentified
  misc_feature 1..23: note = Description of Unknown: Target sequence
  source 1..23: mol_type = unassigned DNA
gctctggctaaagagggaatggg

SEQ ID NO: 149 - DNA, 23 bp, unidentified
  misc_feature 1..23: note = Description of Unknown: Target sequence
  source 1..23: mol_type = unassigned DNA
cggctctggctaaagagggaatg

SEQ ID NO: 150 - DNA, 23 bp, unidentified
  misc_feature 1..23: note = Description of Unknown: Target sequence
  source 1..23: mol_type = unassigned DNA
tcactctcgaagacgctgctcgc

SEQ ID NO: 151 - DNA, 23 bp, unidentified
  misc_feature 1..23: note = Description of Unknown: Target sequence
  source 1..23: mol_type = unassigned DNA
gcttccctgtggtggccgagcgc

SEQ ID NO: 152 - DNA, 23 bp, unidentified
  misc_feature 1..23: note = Description of Unknown: Target sequence
  source 1..23: mol_type = unassigned DNA
agtcccaaatatgtagctgtttg

SEQ ID NO: 153 - DNA, 23 bp, unidentified
  misc_feature 1..23: note = Description of Unknown: Target sequence
  source 1..23: mol_type = unassigned DNA
ccccctttccaaagcccattccc

SEQ ID NO: 154 - DNA, 23 bp, unidentified
  misc_feature 1..23: note = Description of Unknown: Target sequence
  source 1..23: mol_type = unassigned DNA
aagacgctgctcgctccattcac

SEQ ID NO: 155 - DNA, 23 bp, unidentified
  misc_feature 1..23: note = Description of Unknown: Target sequence
  source 1..23: mol_type = unassigned DNA
gtccacctaaccgctgcgcctcc

SEQ ID NO: 156 - DNA, 23 bp, unidentified
  misc_feature 1..23: note = Description of Unknown: Target sequence
  source 1..23: mol_type = unassigned DNA
tggaccccctatttctgacctcc

SEQ ID NO: 157 - DNA, 23 bp, unidentified
  misc_feature 1..23: note = Description of Unknown: Target sequence
  source 1..23: mol_type = unassigned DNA
ggaggcgcagcggttaggtggac

SEQ ID NO: 158 - DNA, 23 bp, unidentified
  misc_feature 1..23: note = Description of Unknown: Target sequence
  source 1..23: mol_type = unassigned DNA
cctatttctgacctcccaaacag

SEQ ID NO: 159 - DNA, 23 bp, unidentified
  misc_feature 1..23: note = Description of Unknown: Target sequence
  source 1..23: mol_type = unassigned DNA
gtcccaaatatgtagctgtttgg

SEQ ID NO: 160 - DNA, 23 bp, unidentified
  misc_feature 1..23: note = Description of Unknown: Target sequence
  source 1..23: mol_type = unassigned DNA
ctagggggcgctcggccaccaca

SEQ ID NO: 161 - DNA, 23 bp, unidentified
  misc_feature 1..23: note = Description of Unknown: Target sequence
  source 1..23: mol_type = unassigned DNA
cctttccaaagcccattccctct

SEQ ID NO: 162 - DNA, 23 bp, unidentified
  misc_feature 1..23: note = Description of Unknown: Target sequence
  source 1..23: mol_type = unassigned DNA
ctccaacgccctcaaccccacac

SEQ ID NO: 163 - DNA, 23 bp, unidentified
  misc_feature 1..23: note = Description of Unknown: Target sequence
  source 1..23: mol_type = unassigned DNA
cacgtaacctcactttcctgctc

SEQ ID NO: 164 - DNA, 23 bp, unidentified
  misc_feature 1..23: note = Description of Unknown: Target sequence
  source 1..23: mol_type = unassigned DNA
ccccaccccctttccaaagccca

SEQ ID NO: 165 - DNA, 23 bp, unidentified
  misc_feature 1..23: note = Description of Unknown: Target sequence
  source 1..23: mol_type = unassigned DNA
gctaaaataaaggaggaggaagc

SEQ ID NO: 166 - DNA, 23 bp, unidentified
  misc_feature 1..23: note = Description of Unknown: Target sequence
  source 1..23: mol_type = unassigned DNA
cccccggaaactctgtccagaga

SEQ ID NO: 167 - DNA, 23 bp, unidentified
  misc_feature 1..23: note = Description of Unknown: Target sequence
  source 1..23: mol_type = unassigned DNA
atagatctgtgtgtccctctccc

SEQ ID NO: 168 - DNA, 23 bp, unidentified
  misc_feature 1..23: note = Description of Unknown: Target sequence
  source 1..23: mol_type = unassigned DNA
gtctccgtgaacgttcccttagc

SEQ ID NO: 169 - DNA, 23 bp, unidentified
  misc_feature 1..23: note = Description of Unknown: Target sequence
  source 1..23: mol_type = unassigned DNA
tggagtgacccctggccttctcc

SEQ ID NO: 170 - DNA, 23 bp, unidentified
  misc_feature 1..23: note = Description of Unknown: Target sequence
  source 1..23: mol_type = unassigned DNA
ctttccaaagcccattccctctt

SEQ ID NO: 171 - DNA, 23 bp, unidentified
  misc_feature 1..23: note = Description of Unknown: Target sequence
  source 1..23: mol_type = unassigned DNA
ggggcggatgggtaattttcagg

SEQ ID NO: 172 - DNA, 23 bp, unidentified
  misc_feature 1..23: note = Description of Unknown: Target sequence
  source 1..23: mol_type = unassigned DNA
cggagactgaacactcctcaaac

SEQ ID NO: 173 - DNA, 23 bp, unidentified
  misc_feature 1..23: note = Description of Unknown: Target sequence
  source 1..23: mol_type = unassigned DNA
cccaccccctttccaaagcccat

SEQ ID NO: 174 - DNA, 23 bp, unidentified
  misc_feature 1..23: note = Description of Unknown: Target sequence
  source 1..23: mol_type = unassigned DNA
ccaccccctttccaaagcccatt

SEQ ID NO: 175 - DNA, 30 bp, synthetic construct
  misc_feature 1..30: note = Description of Artificial Sequence: Synthetic oligonucleotide
  source 1..30: mol_type = other DNA
ccgatggtccatgtctgttactcgcctgtc

SEQ ID NO: 176 - DNA, 23 bp, synthetic construct
  misc_feature 1..23: note = Description of Artificial Sequence: Synthetic oligonucleotide
  source 1..23: mol_type = other DNA
aaattccagcaccgagcgccctg

SEQ ID NO: 177 - DNA, 23 bp, synthetic construct
  misc_feature 1..23: note = Description of Artificial Sequence: Synthetic oligonucleotide
  source 1..23: mol_type = other DNA
aagaaatattacaacatataaaa

SEQ ID NO: 178 - DNA, 23 bp, synthetic construct
  misc_feature 1..23: note = Description of Artificial Sequence: Synthetic oligonucleotide
  source 1..23: mol_type = other DNA
gtcacccctgtttctggcaccag

SEQ ID NO: 179 - DNA, 23 bp, synthetic construct
  misc_feature 1..23: note = Description of Artificial Sequence: Synthetic oligonucleotide
  source 1..23: mol_type = other DNA
tggtgccagaaacaggggtgacg

SEQ ID NO: 180 - DNA, 24 bp, synthetic construct
  misc_feature 1..24: note = Description of Artificial Sequence: Synthetic oligonucleotide
  source 1..24: mol_type = other DNA
gagaagtcatttaataaggccact

SEQ ID NO: 181 - DNA, 23 bp, synthetic construct
  misc_feature 1..23: note = Description of Artificial Sequence: Synthetic oligonucleotide
  source 1..23: mol_type = other DNA
gcagttgtcgcagttttacaacc

SEQ ID NO: 182 - DNA, 23 bp, synthetic construct
  misc_feature 1..23: note = Description of Artificial Sequence: Synthetic oligonucleotide
  source 1..23: mol_type = other DNA
acccggataacaaggaggaacgc

SEQ ID NO: 183 - DNA, 23 bp, synthetic construct
  misc_feature 1..23: note = Description of Artificial Sequence: Synthetic oligonucleotide
  source 1..23: mol_type = other DNA
gagttgattggattgagaataga

SEQ ID NO: 184 - DNA, 23 bp, synthetic construct
  misc_feature 1..23: note = Description of Artificial Sequence: Synthetic oligonucleotide
  source 1..23: mol_type = other DNA
gcctctccctgctcagaatctgg

SEQ ID NO: 185 - DNA, 23 bp, synthetic construct
  misc_feature 1..23: note = Description of Artificial Sequence: Synthetic oligonucleotide
  source 1..23: mol_type = other DNA
tagctgtttgggaggtcagaaat

SEQ ID NO: 186 - DNA, 23 bp, synthetic construct
  misc_feature 1..23: note = Description of Artificial Sequence: Synthetic oligonucleotide
  source 1..23: mol_type = other DNA
gacatgtcccatttgtgggaact

SEQ ID NO: 187 - DNA, 23 bp, synthetic construct
  misc_feature 1..23: note = Description of Artificial Sequence: Synthetic oligonucleotide
  source 1..23: mol_type = other DNA
ttcgggtgctgtgaacttccctc

SEQ ID NO: 188 - DNA, 23 bp, synthetic construct
  misc_feature 1..23: note = Description of Artificial Sequence: Synthetic oligonucleotide
  source 1..23: mol_type = other DNA
acccactgcgtgggttcccatga

SEQ ID NO: 189 - DNA, 23 bp, synthetic construct
  misc_feature 1..23: note = Description of Artificial Sequence: Synthetic oligonucleotide
  source 1..23: mol_type = other DNA
ccaagtcaaacttctcttcagtc

SEQ ID NO: 190 - DNA, 23 bp, synthetic construct
  misc_feature 1..23: note = Description of Artificial Sequence: Synthetic oligonucleotide
  source 1..23: mol_type = other DNA
ccctttaggacacatgctgtcta

SEQ ID NO: 191 - DNA, 23 bp, synthetic construct
  misc_feature 1..23: note = Description of Artificial Sequence: Synthetic oligonucleotide
  source 1..23: mol_type = other DNA
agtgcaccttcggcgtgctgcag

SEQ ID NO: 192 - DNA, 23 bp, synthetic construct
  misc_feature 1..23: note = Description of Artificial Sequence: Synthetic oligonucleotide
  source 1..23: mol_type = other DNA
cccaccatgacaggaagaacggc

SEQ ID NO: 193 - DNA, 23 bp, synthetic construct
  misc_feature 1..23: note = Description of Artificial Sequence: Synthetic oligonucleotide
  source 1..23: mol_type = other DNA
aggcgcttccccagcacaaactg

SEQ ID NO: 194 - DNA, 23 bp, synthetic construct
  misc_feature 1..23: note = Description of Artificial Sequence: Synthetic oligonucleotide
  source 1..23: mol_type = other DNA
gcgatgttttttctggagattta

SEQ ID NO: 195 - DNA, 23 bp, synthetic construct
  misc_feature 1..23: note = Description of Artificial Sequence: Synthetic oligonucleotide
  source 1..23: mol_type = other DNA
gctaaaataaaggaggaggaagc

SEQ ID NO: 196 - DNA, 23 bp, synthetic construct
  misc_feature 1..23: note = Description of Artificial Sequence: Synthetic oligonucleotide
  source 1..23: mol_type = other DNA
gtctccgtgaacgttcccttagc

SEQ ID NO: 197 - DNA, 23 bp, synthetic construct
  misc_feature 1..23: note = Description of Artificial Sequence: Synthetic oligonucleotide
  source 1..23: mol_type = other DNA
cggagactgaacactcctcaaac

SEQ ID NO: 198 - DNA, 23 bp, synthetic construct
  misc_feature 1..23: note = Description of Artificial Sequence: Synthetic oligonucleotide
  source 1..23: mol_type = other DNA
tggcaatgcgccaccggttgatg

SEQ ID NO: 199 - DNA, 23 bp, synthetic construct
  misc_feature 1..23: note = Description of Artificial Sequence: Synthetic oligonucleotide
  source 1..23: mol_type = other DNA
ctgtggtggccgagcgcccccta

SEQ ID NO: 200 - DNA, 23 bp, synthetic construct
  misc_feature 1..23: note = Description of Artificial Sequence: Synthetic oligonucleotide
  source 1..23: mol_type = other DNA
gtcccaaatatgtagctgtttgg

SEQ ID NO: 201 - DNA, 23 bp, synthetic construct
  misc_feature 1..23: note = Description of Artificial Sequence: Synthetic oligonucleotide
  source 1..23: mol_type = other DNA
cacgtaacctcactttcctgctc

SEQ ID NO: 202 - DNA, 23 bp, synthetic construct
  misc_feature 1..23: note = Description of Artificial Sequence: Synthetic oligonucleotide
  source 1..23: mol_type = other DNA
tctttagccagagccggggtgtg

SEQ ID NO: 203 - DNA, 23 bp, synthetic construct
  misc_feature 1..23: note = Description of Artificial Sequence: Synthetic oligonucleotide
  source 1..23: mol_type = other DNA
cccccggaaactctgtccagaga

SEQ ID NO: 204 - DNA, 23 bp, synthetic construct
  misc_feature 1..23: note = Description of Artificial Sequence: Synthetic oligonucleotide
  source 1..23: mol_type = other DNA
ggggcggatgggtaattttcagg

SEQ ID NO: 205 - DNA, 23 bp, synthetic construct
  misc_feature 1..23: note = Description of Artificial Sequence: Synthetic oligonucleotide
  source 1..23: mol_type = other DNA
atagatctgtgtgtccctctccc

SEQ ID NO: 206 - DNA, 23 bp, synthetic construct
  misc_feature 1..23: note = Description of Artificial Sequence: Synthetic oligonucleotide
  source 1..23: mol_type = other DNA
aaagcccattccctctttagcca

SEQ ID NO: 207 - DNA, 23 bp, synthetic construct
  misc_feature 1..23: note = Description of Artificial Sequence: Synthetic oligonucleotide
  source 1..23: mol_type = other DNA
cccaccccctttccaaagcccat

SEQ ID NO: 208 - DNA, 23 bp, synthetic construct
  misc_feature 1..23: note = Description of Artificial Sequence: Synthetic oligonucleotide
  source 1..23: mol_type = other DNA
aaaattttacaccacaaaatgtt

SEQ ID NO: 209 - DNA, 23 bp, synthetic construct
  misc_feature 1..23: note = Description of Artificial Sequence: Synthetic oligonucleotide
  source 1..23: mol_type = other DNA
aagatgatattttctttaatggt

SEQ ID NO: 210 - DNA, 23 bp, synthetic construct
  misc_feature 1..23: note = Description of Artificial Sequence: Synthetic oligonucleotide
  source 1..23: mol_type = other DNA
ttaaagaaaatatcatctttggt

SEQ ID NO: 211 - DNA, 23 bp, synthetic construct
  misc_feature 1..23: note = Description of Artificial Sequence: Synthetic oligonucleotide
  source 1..23: mol_type = other DNA
taaactcattaatgcccttcggc

SEQ ID NO: 212 - DNA, 23 bp, synthetic construct
  misc_feature 1..23: note = Description of Artificial Sequence: Synthetic oligonucleotide
  source 1..23: mol_type = other DNA
aggaaaactgagaacagaatgaa

SEQ ID NO: 213 - DNA, 23 bp, synthetic construct
  misc_feature 1..23: note = Description of Artificial Sequence: Synthetic oligonucleotide
  source 1..23: mol_type = other DNA
catcaaccggtggcgcattgcca

SEQ ID NO: 214 - DNA, 23 bp, synthetic construct
  misc_feature 1..23: note = Description of Artificial Sequence: Synthetic oligonucleotide
  source 1..23: mol_type = other DNA
tccccattggcctgcttcgtggc

SEQ ID NO: 215 - DNA, 23 bp, synthetic construct
  misc_feature 1..23: note = Description of Artificial Sequence: Synthetic oligonucleotide
  source 1..23: mol_type = other DNA
ggcttcaagccctgtggggccat

SEQ ID NO: 216 - DNA, 23 bp, synthetic construct
  misc_feature 1..23: note = Description of Artificial Sequence: Synthetic oligonucleotide
  source 1..23: mol_type = other DNA
atgtcacctccaatgactagggt

SEQ ID NO: 217 - DNA, 23 bp, synthetic construct
  misc_feature 1..23: note = Description of Artificial Sequence: Synthetic oligonucleotide
  source 1..23: mol_type = other DNA
atgtcctccccattggcctgctt

SEQ ID NO: 218 - DNA, 23 bp, synthetic construct
  misc_feature 1..23: note = Description of Artificial Sequence: Synthetic oligonucleotide
  source 1..23: mol_type = other DNA
ttccctctttagccagagccggg

SEQ ID NO: 219 - DNA, 23 bp, synthetic construct
  misc_feature 1..23: note = Description of Artificial Sequence: Synthetic oligonucleotide
  source 1..23: mol_type = other DNA
gccaccacagggaagctgggtga

SEQ ID NO: 220 - DNA, 23 bp, synthetic construct
  misc_feature 1..23: note = Description of Artificial Sequence: Synthetic oligonucleotide
  source 1..23: mol_type = other DNA
caaatatgtagctgtttgggagg

SEQ ID NO: 221 - DNA, 23 bp, synthetic construct
  misc_feature 1..23: note = Description of Artificial Sequence: Synthetic oligonucleotide
  source 1..23: mol_type = other DNA
agcgccccctagtgactgccgtc

SEQ ID NO: 222 - DNA, 23 bp, synthetic construct
  misc_feature 1..23: note = Description of Artificial Sequence: Synthetic oligonucleotide
  source 1..23: mol_type = other DNA
attccctctttagccagagccgg

SEQ ID NO: 223 - DNA, 23 bp, synthetic construct
  misc_feature 1..23: note = Description of Artificial Sequence: Synthetic oligonucleotide
  source 1..23: mol_type = other DNA
gctctggctaaagagggaatggg

SEQ ID NO: 224 - DNA, 23 bp, synthetic construct
  misc_feature 1..23: note = Description of Artificial Sequence: Synthetic oligonucleotide
  source 1..23: mol_type = other DNA
gagccggggtgtgcagacggcag

SEQ ID NO: 225 - DNA, 23 bp, synthetic construct
  misc_feature 1..23: note = Description of Artificial Sequence: Synthetic oligonucleotide
  source 1..23: mol_type = other DNA
ctccattcacccagcttccctgt

SEQ ID NO: 226 - DNA, 23 bp, synthetic construct
  misc_feature 1..23: note = Description of Artificial Sequence: Synthetic oligonucleotide
  source 1..23: mol_type = other DNA
gaaatagggggtccaggagcaaa

SEQ ID NO: 227 - DNA, 23 bp, synthetic construct
  misc_feature 1..23: note = Description of Artificial Sequence: Synthetic oligonucleotide
  source 1..23: mol_type = other DNA
agtcccaaatatgtagctgtttg

SEQ ID NO: 228 - DNA, 23 bp, synthetic construct
  misc_feature 1..23: note = Description of Artificial Sequence: Synthetic oligonucleotide
  source 1..23: mol_type = other DNA
tgggctctctgtacatgaagcaa

SEQ ID NO: 229 - DNA, 23 bp, synthetic construct
  misc_feature 1..23: note = Description of Artificial Sequence: Synthetic oligonucleotide
  source 1..23: mol_type = other DNA
cagggaagctgggtgaatggagc

SEQ ID NO: 230 - DNA, 23 bp, synthetic construct
  misc_feature 1..23: note = Description of Artificial Sequence: Synthetic oligonucleotide
  source 1..23: mol_type = other DNA
cggctctggctaaagagggaatg

SEQ ID NO: 231 - DNA, 23 bp, synthetic construct
  misc_feature 1..23: note = Description of Artificial Sequence: Synthetic oligonucleotide
  source 1..23: mol_type = other DNA
gcttccctgtggtggccgagcgc

SEQ ID NO: 232 - DNA, 23 bp, synthetic construct
  misc_feature 1..23: note = Description of Artificial Sequence: Synthetic oligonucleotide
  source 1..23: mol_type = other DNA
tctgcacaccccggctctggcta

SEQ ID NO: 233 - DNA, 23 bp, synthetic construct
  misc_feature 1..23: note = Description of Artificial Sequence: Synthetic oligonucleotide
  source 1..23: mol_type = other DNA
cctagtgactgccgtctgcacac

SEQ ID NO: 234 - DNA, 23 bp, synthetic construct
  misc_feature 1..23: note = Description of Artificial Sequence: Synthetic oligonucleotide
  source 1..23: mol_type = other DNA
cctatttctgacctcccaaacag

SEQ ID NO: 235 - DNA, 23 bp, synthetic construct
  misc_feature 1..23: note = Description of Artificial Sequence: Synthetic oligonucleotide
  source 1..23: mol_type = other DNA
ccacagggaagctgggtgaatgg

SEQ ID NO: 236 - DNA, 23 bp, synthetic construct
  misc_feature 1..23: note = Description of Artificial Sequence: Synthetic oligonucleotide
  source 1..23: mol_type = other DNA
tcactctcgaagacgctgctcgc

SEQ ID NO: 237 - DNA, 23 bp, synthetic construct
  misc_feature 1..23: note = Description of Artificial Sequence: Synthetic oligonucleotide
  source 1..23: mol_type = other DNA
ctagggggcgctcggccaccaca

SEQ ID NO: 238 - DNA, 23 bp, synthetic construct
  misc_feature 1..23: note = Description of Artificial Sequence: Synthetic oligonucleotide
  source 1..23: mol_type = other DNA
gggtgtgcagacggcagtcacta

SEQ ID NO: 239 - DNA, 23 bp, synthetic construct
  misc_feature 1..23: note = Description of Artificial Sequence: Synthetic oligonucleotide
  source 1..23: mol_type = other DNA
aagacgctgctcgctccattcac

SEQ ID NO: 240 - DNA, 23 bp, synthetic construct
  misc_feature 1..23: note = Description of Artificial Sequence: Synthetic oligonucleotide
  source 1..23: mol_type = other DNA
ctccaacgccctcaaccccacac

SEQ ID NO: 241 - DNA, 23 bp, synthetic construct
  misc_feature 1..23: note = Description of Artificial Sequence: Synthetic oligonucleotide
  source 1..23: mol_type = other DNA
tggaccccctatttctgacctcc

SEQ ID NO: 242 - DNA, 23 bp, synthetic construct
  misc_feature 1..23: note = Description of Artificial Sequence: Synthetic oligonucleotide
  source 1..23: mol_type = other DNA
tggagtgacccctggccttctcc

SEQ ID NO: 243 - DNA, 23 bp, synthetic construct
  misc_feature 1..23: note = Description of Artificial Sequence: Synthetic oligonucleotide
  source 1..23: mol_type = other DNA
cctttccaaagcccattccctct

SEQ ID NO: 244 - DNA, 23 bp, synthetic construct
  misc_feature 1..23: note = Description of Artificial Sequence: Synthetic oligonucleotide
  source 1..23: mol_type = other DNA
ccaccccctttccaaagcccatt

SEQ ID NO: 245 - DNA, 23 bp, synthetic construct
  misc_feature 1..23: note = Description of Artificial Sequence: Synthetic oligonucleotide
  source 1..23: mol_type = other DNA
ctaggaatattgaagggggcagg

SEQ ID NO: 246 - DNA, 23 bp, synthetic construct
  misc_feature 1..23: note = Description of Artificial Sequence: Synthetic oligonucleotide
  source 1..23: mol_type = other DNA
gtgctcaatgaaaggagataagg

SEQ ID NO: 247 - DNA, 23 bp, synthetic construct
  misc_feature 1..23: note = Description of Artificial Sequence: Synthetic oligonucleotide
  source 1..23: mol_type = other DNA
tcctccggttctggaaccacacc

SEQ ID NO: 248 - DNA, 23 bp, synthetic construct
  misc_feature 1..23: note = Description of Artificial Sequence: Synthetic oligonucleotide
  source 1..23: mol_type = other DNA
gggtgatcagacccaacagcagg

SEQ ID NO: 249 - DNA, 23 bp, synthetic construct
  misc_feature 1..23: note = Description of Artificial Sequence: Synthetic oligonucleotide
  source 1..23: mol_type = other DNA
atggtgccaggcataatccagga

SEQ ID NO: 250 - DNA, 23 bp, synthetic construct
  misc_feature 1..23: note = Description of Artificial Sequence: Synthetic oligonucleotide
  source 1..23: mol_type = other DNA
ccttcagctaaaataaaggagga

SEQ ID NO: 251 - DNA, 23 bp, synthetic construct
  misc_feature 1..23: note = Description of Artificial Sequence: Synthetic oligonucleotide
  source 1..23: mol_type = other DNA
aggagtgttcagtctccgtgaac

SEQ ID NO: 252 - DNA, 23 bp, synthetic construct
  misc_feature 1..23: note = Description of Artificial Sequence: Synthetic oligonucleotide
  source 1..23: mol_type = other DNA
ctgatggtccatgtctgttactc

SEQ ID NO: 253 - DNA, 23 bp, synthetic construct
  misc_feature 1..23: note = Description of Artificial Sequence: Synthetic oligonucleotide
  source 1..23: mol_type = other DNA
gctgaagggaaataaaaggaaaa

SEQ ID NO: 254 - DNA, 23 bp, synthetic construct
  misc_feature 1..23: note = Description of Artificial Sequence: Synthetic oligonucleotide
  source 1..23: mol_type = other DNA
gggaggcctggagtcatggcccc

SEQ ID NO: 255 - DNA, 23 bp, synthetic construct
  misc_feature 1..23: note = Description of Artificial Sequence: Synthetic oligonucleotide
  source 1..23: mol_type = other DNA
tggttgcccaccctagtcattgg

SEQ ID NO: 256 - DNA, 23 bp, synthetic construct
  misc_feature 1..23: note = Description of Artificial Sequence: Synthetic oligonucleotide
  source 1..23: mol_type = other DNA
gccagagccggggtgtgcagacg

SEQ ID NO: 257 - DNA, 23 bp, synthetic construct
  misc_feature 1..23: note = Description of Artificial Sequence: Synthetic oligonucleotide
  source 1..23: mol_type = other DNA
caaagcccattccctctttagcc

SEQ ID NO: 258 - DNA, 23 bp, synthetic construct
  misc_feature 1..23: note = Description of Artificial Sequence: Synthetic oligonucleotide
  source 1..23: mol_type = other DNA
gtcccaggaggatggcctggctg

SEQ ID NO: 259 - DNA, 23 bp, synthetic construct
  misc_feature 1..23: note = Description of Artificial Sequence: Synthetic oligonucleotide
  source 1..23: mol_type = other DNA
aggaggatggcctggctgatgag

SEQ ID NO: 260 - DNA, 23 bp, synthetic construct
  misc_feature 1..23: note = Description of Artificial Sequence: Synthetic oligonucleotide
  source 1..23: mol_type = other DNA
atctgtagcctctgggtctcctc

SEQ ID NO: 261 - DNA, 23 bp, synthetic construct
  misc_feature 1..23: note = Description of Artificial Sequence: Synthetic oligonucleotide
  source 1..23: mol_type = other DNA
tggcttcttggtgaagatgagca

SEQ ID NO: 262 - DNA, 23 bp, synthetic construct
  misc_feature 1..23: note = Description of Artificial Sequence: Synthetic oligonucleotide
  source 1..23: mol_type = other DNA
tcaatgtactccacatggggcaa

SEQ ID NO: 263 - DNA, 23 bp, synthetic construct
  misc_feature 1..23: note = Description of Artificial Sequence: Synthetic oligonucleotide
  source 1..23: mol_type = other DNA
tgggatgctctgggcgaagacaa

SEQ ID NO: 264 - DNA, 23 bp, synthetic construct
  misc_feature 1..23: note = Description of Artificial Sequence: Synthetic oligonucleotide
  source 1..23: mol_type = other DNA
gatgggcaccctggatgctggta

SEQ ID NO: 265 - DNA, 23 bp, synthetic construct
  misc_feature 1..23: note = Description of Artificial Sequence: Synthetic oligonucleotide
  source 1..23: mol_type = other DNA
ggccgctgaccacacctgccagg

SEQ ID NO: 266 - DNA, 23 bp, synthetic construct
  misc_feature 1..23: note = Description of Artificial Sequence: Synthetic oligonucleotide
  source 1..23: mol_type = other DNA
gatgggcacccactgctctgcgt

SEQ ID NO: 267 - DNA, 23 bp, synthetic construct
  misc_feature 1..23: note = Description of Artificial Sequence: Synthetic oligonucleotide
  source 1..23: mol_type = other DNA
ttcaatctgtagcctctgggtct

SEQ ID NO: 268 - DNA, 23 bp, synthetic construct
  misc_feature 1..23: note = Description of Artificial Sequence: Synthetic oligonucleotide
  source 1..23: mol_type = other DNA
tgacctcttccctggcttcttgg

SEQ ID NO: 269 - DNA, 23 bp, synthetic construct
  misc_feature 1..23: note = Description of Artificial Sequence: Synthetic oligonucleotide
  source 1..23: mol_type = other DNA
tcttcgcccagagcatcccatgg

SEQ ID NO: 270 - DNA, 23 bp, synthetic construct
  misc_feature 1..23: note = Description of Artificial Sequence: Synthetic oligonucleotide
  source 1..23: mol_type = other DNA
ggagagatttatttgaagaaata

SEQ ID NO: 271 - DNA, 23 bp, synthetic construct
  misc_feature 1..23: note = Description of Artificial Sequence: Synthetic oligonucleotide
  source 1..23: mol_type = other DNA
atggccgcttggagccaatcgtg

SEQ ID NO: 272 - DNA, 23 bp, synthetic construct
  misc_feature 1..23: note = Description of Artificial Sequence: Synthetic oligonucleotide
  source 1..23: mol_type = other DNA
acgatcttcaccgcataatcaga

SEQ ID NO: 273 - DNA, 23 bp, synthetic construct
  misc_feature 1..23: note = Description of Artificial Sequence: Synthetic oligonucleotide
  source 1..23: mol_type = other DNA
cccaaattccacattgtcgctgc

SEQ ID NO: 274 - DNA, 23 bp, synthetic construct
  misc_feature 1..23: note = Description of Artificial Sequence: Synthetic oligonucleotide
  source 1..23: mol_type = other DNA
cactatgaccttcagaaaggcat

SEQ ID NO: 275 - DNA, 23 bp, synthetic construct
  misc_feature 1..23: note = Description of Artificial Sequence: Synthetic oligonucleotide
  source 1..23: mol_type = other DNA
tcacctgcagggcagcactcttg

SEQ ID NO: 276 - DNA, 23 bp, synthetic construct
  misc_feature 1..23: note = Description of Artificial Sequence: Synthetic oligonucleotide
  source 1..23: mol_type = other DNA
acgtctcttcggttatccagaag

SEQ ID NO: 277 - DNA, 23 bp, synthetic construct
  misc_feature 1..23: note = Description of Artificial Sequence: Synthetic oligonucleotide
  source 1..23: mol_type = other DNA
ttcgaaatgttagatatcgttat

SEQ ID NO: 278 - DNA, 23 bp, synthetic construct
  misc_feature 1..23: note = Description of Artificial Sequence: Synthetic oligonucleotide
  source 1..23: mol_type = other DNA
atgcaggcatcacgaatggccag

SEQ ID NO: 279 - DNA, 23 bp, synthetic construct
  misc_feature 1..23: note = Description of Artificial Sequence: Synthetic oligonucleotide
  source 1..23: mol_type = other DNA
ctgaatggaattcgtttatatgg

SEQ ID NO: 280 - DNA, 23 bp, synthetic construct
  misc_feature 1..23: note = Description of Artificial Sequence: Synthetic oligonucleotide
  source 1..23: mol_type = other DNA
aggctctgcaactcctgccgtag

SEQ ID NO: 281 - DNA, 23 bp, synthetic construct
  misc_feature 1..23: note = Description of Artificial Sequence: Synthetic oligonucleotide
  source 1..23: mol_type = other DNA
cgtgtgacacgcagaagggtacc

SEQ ID NO: 282 - DNA, 23 bp, synthetic construct
  misc_feature 1..23: note = Description of Artificial Sequence: Synthetic oligonucleotide
  source 1..23: mol_type = other DNA
acatttgcttctctttaccatag

SEQ ID NO: 283 - DNA, 23 bp, synthetic construct
  misc_feature 1..23: note = Description of Artificial Sequence: Synthetic oligonucleotide
  source 1..23: mol_type = other DNA
tcctggagaccctccagccgcag

SEQ ID NO: 284 - DNA, 23 bp, synthetic construct
  misc_feature 1..23: note = Description of Artificial Sequence: Synthetic oligonucleotide
  source 1..23: mol_type = other DNA
cagttcgcggctctccacgtcaa

SEQ ID NO: 285 - DNA, 23 bp, synthetic construct
  misc_feature 1..23: note = Description of Artificial Sequence: Synthetic oligonucleotide
  source 1..23: mol_type = other DNA
agtggatatttctgttgccacat

SEQ ID NO: 286 - DNA, 23 bp, synthetic construct
  misc_feature 1..23: note = Description of Artificial Sequence: Synthetic oligonucleotide
  source 1..23: mol_type = other DNA
tggaaggacatcttccacaagaa

SEQ ID NO: 287 - DNA, 23 bp, synthetic construct
  misc_feature 1..23: note = Description of Artificial Sequence: Synthetic oligonucleotide
  source 1..23: mol_type = other DNA
ctctgctgttgcccagccacaca

SEQ ID NO: 288 - DNA, 23 bp, synthetic construct
  misc_feature 1..23: note = Description of Artificial Sequence: Synthetic oligonucleotide
  source 1..23: mol_type = other DNA
ccagtccagtcataacgcttagg

SEQ ID NO: 289 - DNA, 23 bp, synthetic construct
  misc_feature 1..23: note = Description of Artificial Sequence: Synthetic oligonucleotide
  source 1..23: mol_type = other DNA
ggtcctgtctatatgtgacttca

SEQ ID NO: 290 - DNA, 23 bp, synthetic construct
  misc_feature 1..23: note = Description of Artificial Sequence: Synthetic oligonucleotide
  source 1..23: mol_type = other DNA
cagaacactgtatgctgccatca

SEQ ID NO: 291 - DNA, 23 bp, synthetic construct
  misc_feature 1..23: note = Description of Artificial Sequence: Synthetic oligonucleotide
  source 1..23: mol_type = other DNA
cctgagagctgggccgaacgggg

SEQ ID NO: 292 - DNA, 23 bp, synthetic construct
  misc_feature 1..23: note = Description of Artificial Sequence: Synthetic oligonucleotide
  source 1..23: mol_type = other DNA
cccttggcattgctgatcttcag

SEQ ID NO: 293 - DNA, 23 bp, synthetic construct
  misc_feature 1..23: note = Description of Artificial Sequence: Synthetic oligonucleotide
  source 1..23: mol_type = other DNA
cggtcttatctatgaggagactc

SEQ ID NO: 294 - DNA, 23 bp, synthetic construct
  misc_feature 1..23: note = Description of Artificial Sequence: Synthetic oligonucleotide
  source 1..23: mol_type = other DNA
agcggccatcaaacatatctgcc

SEQ ID NO: 295 - DNA, 23 bp, synthetic construct
  misc_feature 1..23: note = Description of Artificial Sequence: Synthetic oligonucleotide
  source 1..23: mol_type = other DNA
ccgcataatcagagatactggaa

SEQ ID NO: 296 - DNA, 23 bp, synthetic construct
  misc_feature 1..23: note = Description of Artificial Sequence: Synthetic oligonucleotide
  source 1..23: mol_type = other DNA
aaattccacattgtcgctgcagc

SEQ ID NO: 297 - DNA, 23 bp, synthetic construct
  misc_feature 1..23: note = Description of Artificial Sequence: Synthetic oligonucleotide
  source 1..23: mol_type = other DNA
acccaaatgcctttctgaaggtc

SEQ ID NO: 298 - DNA, 23 bp, synthetic construct
  misc_feature 1..23: note = Description of Artificial Sequence: Synthetic oligonucleotide
  source 1..23: mol_type = other DNA
tgcgtgatctgctttgtcacctg

SEQ ID NO: 299 - DNA, 23 bp, synthetic construct
  misc_feature 1..23: note = Description of Artificial Sequence: Synthetic oligonucleotide
  source 1..23: mol_type = other DNA
agcgcctgaggctggtggcaggc

SEQ ID NO: 300 - DNA, 23 bp, synthetic construct
  misc_feature 1..23: note = Description of Artificial Sequence: Synthetic oligonucleotide
  source 1..23: mol_type = other DNA
aaatgttagatatcgttatcaac

SEQ ID NO: 301 - DNA, 23 bp, synthetic construct
  misc_feature 1..23: note = Description of Artificial Sequence: Synthetic oligonucleotide
  source 1..23: mol_type = other DNA
gtttgatgcaggcatcacgaatg

SEQ ID NO: 302 - DNA, 23 bp, synthetic construct
  misc_feature 1..23: note = Description of Artificial Sequence: Synthetic oligonucleotide
  source 1..23: mol_type = other DNA
tttatatggaagaccaattaacg

SEQ ID NO: 303 - DNA, 23 bp, synthetic construct
  misc_feature 1..23: note = Description of Artificial Sequence: Synthetic oligonucleotide
  source 1..23: mol_type = other DNA
ggctctgcaactcctgccgtagc

SEQ ID NO: 304 - DNA, 23 bp, synthetic construct
  misc_feature 1..23: note = Description of Artificial Sequence: Synthetic oligonucleotide
  source 1..23: mol_type = other DNA
gcgggacagcagtgtatgtggtc

SEQ ID NO: 305 - DNA, 23 bp, synthetic construct
  misc_feature 1..23: note = Description of Artificial Sequence: Synthetic oligonucleotide
  source 1..23: mol_type = other DNA
tatggtaaagagaagcaaatgtg

SEQ ID NO: 306 - DNA, 23 bp, synthetic construct
  misc_feature 1..23: note = Description of Artificial Sequence: Synthetic oligonucleotide
  source 1..23: mol_type = other DNA
gggagggcatggagtagaccaag

SEQ ID NO: 307 - DNA, 23 bp, synthetic construct
  misc_feature 1..23: note = Description of Artificial Sequence: Synthetic oligonucleotide
  source 1..23: mol_type = other DNA
agttcgcggctctccacgtcaaa

SEQ ID NO: 308 - DNA, 23 bp, synthetic construct
  misc_feature 1..23: note = Description of Artificial Sequence: Synthetic oligonucleotide
  source 1..23: mol_type = other DNA
aggtctctttcagtggatatttc

SEQ ID NO: 309 - DNA, 23 bp, synthetic construct
  misc_feature 1..23: note = Description of Artificial Sequence: Synthetic oligonucleotide
  source 1..23: mol_type = other DNA
acaagaacaaccagctggctctc

SEQ ID NO: 310 - DNA, 23 bp, synthetic construct
  misc_feature 1..23: note = Description of Artificial Sequence: Synthetic oligonucleotide
  source 1..23: mol_type = other DNA
tctgctgttgcccagccacacat

SEQ ID NO: 311 - DNA, 23 bp, synthetic construct
  misc_feature 1..23: note = Description of Artificial Sequence: Synthetic oligonucleotide
  source 1..23: mol_type = other DNA
agtccagtcataacgcttaggtc

SEQ ID NO: 312 - DNA, 23 bp, synthetic construct
  misc_feature 1..23: note = Description of Artificial Sequence: Synthetic oligonucleotide
  source 1..23: mol_type = other DNA
tgaagtcacatatagacaggacc

SEQ ID NO: 313 - DNA, 23 bp, synthetic construct
  misc_feature 1..23: note = Description of Artificial Sequence: Synthetic oligonucleotide
  source 1..23: mol_type = other DNA
gaacactgtatgctgccatcaaa

SEQ ID NO: 314 - DNA, 23 bp, synthetic construct
  misc_feature 1..23: note = Description of Artificial Sequence: Synthetic oligonucleotide
  source 1..23: mol_type = other DNA
gcccagctctcagggaaacgaag

SEQ ID NO: 315 - DNA, 23 bp, synthetic construct
  misc_feature 1..23: note = Description of Artificial Sequence: Synthetic oligonucleotide
  source 1..23: mol_type = other DNA
tttacccttggcattgctgatct

SEQ ID NO: 316 - DNA, 23 bp, synthetic construct
  misc_feature 1..23: note = Description of Artificial Sequence: Synthetic oligonucleotide
  source 1..23: mol_type = other DNA
ggtcttatctatgaggagactcg

SEQ ID NO: 317 - DNA, 23 bp, synthetic construct
  misc_feature 1..23: note = Description of Artificial Sequence: Synthetic oligonucleotide
  source 1..23: mol_type = other DNA
tgccattacctctgtcgccttgc

SEQ ID NO: 318 - DNA, 23 bp, synthetic construct
  misc_feature 1..23: note = Description of Artificial Sequence: Synthetic oligonucleotide
  source 1..23: mol_type = other DNA
tctgattatgcggtgaagatcgt

SEQ ID NO: 319 - DNA, 23 bp, synthetic construct
  misc_feature 1..23: note = Description of Artificial Sequence: Synthetic oligonucleotide
  source 1..23: mol_type = other DNA
taggaggccatggctggatctgg

SEQ ID NO: 320 - DNA, 23 bp, synthetic construct
  misc_feature 1..23: note = Description of Artificial Sequence: Synthetic oligonucleotide
  source 1..23: mol_type = other DNA
tgggtctgctaacagactggggt

SEQ ID NO: 321 - DNA, 23 bp, synthetic construct
  misc_feature 1..23: note = Description of Artificial Sequence: Synthetic oligonucleotide
  source 1..23: mol_type = other DNA
aaggctgctgccaagagtgctgc

SEQ ID NO: 322 - DNA, 23 bp, synthetic construct
  misc_feature 1..23: note = Description of Artificial Sequence: Synthetic oligonucleotide
  source 1..23: mol_type = other DNA
cagaagaacctgcgcttctccca

SEQ ID NO: 323 - DNA, 23 bp, synthetic construct
  misc_feature 1..23: note = Description of Artificial Sequence: Synthetic oligonucleotide
  source 1..23: mol_type = other DNA
taacatttcgaagaaactttgct

SEQ ID NO: 324 - DNA, 23 bp, synthetic construct
  misc_feature 1..23: note = Description of Artificial Sequence: Synthetic oligonucleotide
  source 1..23: mol_type = other DNA
agctactggccattcgtgatgcc

SEQ ID NO: 325 - DNA, 23 bp, synthetic construct
  misc_feature 1..23: note = Description of Artificial Sequence: Synthetic oligonucleotide
  source 1..23: mol_type = other DNA
ccatagctttgctgaatggaatt

SEQ ID NO: 326 - DNA, 23 bp, synthetic construct
  misc_feature 1..23: note = Description of Artificial Sequence: Synthetic oligonucleotide
  source 1..23: mol_type = other DNA
ccaacaagctacggcaggagttg

SEQ ID NO: 327 - DNA, 23 bp, synthetic construct
  misc_feature 1..23: note = Description of Artificial Sequence: Synthetic oligonucleotide
  source 1..23: mol_type = other DNA
tggtcctcacagcacacagccta

SEQ ID NO: 328 - DNA, 23 bp, synthetic construct
  misc_feature 1..23: note = Description of Artificial Sequence: Synthetic oligonucleotide
  source 1..23: mol_type = other DNA
gtaaagagaagcaaatgtgaaac

SEQ ID NO: 329 - DNA, 23 bp, synthetic construct
  misc_feature 1..23: note = Description of Artificial Sequence: Synthetic oligonucleotide
  source 1..23: mol_type = other DNA
cttggtctactccatgccctccc

SEQ ID NO: 330 - DNA, 23 bp, synthetic construct
  misc_feature 1..23: note = Description of Artificial Sequence: Synthetic oligonucleotide
  source 1..23: mol_type = other DNA
ttccgtaacgtggaagttttgat

SEQ ID NO: 331 - DNA, 23 bp, synthetic construct
  misc_feature 1..23: note = Description of Artificial Sequence: Synthetic oligonucleotide
  source 1..23: mol_type = other DNA
cactgaaagagacctggggcagt

SEQ ID NO: 332 - DNA, 23 bp, synthetic construct
  misc_feature 1..23: note = Description of Artificial Sequence: Synthetic oligonucleotide
  source 1..23: mol_type = other DNA
agtgtgagagccagctggttgtt

SEQ ID NO: 333 - DNA, 23 bp, synthetic construct
  misc_feature 1..23: note = Description of Artificial Sequence: Synthetic oligonucleotide
  source 1..23: mol_type = other DNA
atgtgtggctgggcaacagcaga

SEQ ID NO: 334 - DNA, 23 bp, synthetic construct
  misc_feature 1..23: note = Description of Artificial Sequence: Synthetic oligonucleotide
  source 1..23: mol_type = other DNA
actggactgggaaaaactgggtg

SEQ ID NO: 335 - DNA, 23 bp, synthetic construct
  misc_feature 1..23: note = Description of Artificial Sequence: Synthetic oligonucleotide
  source 1..23: mol_type = other DNA
tgtgacttcagggaagactggca

SEQ ID NO: 336 - DNA, 23 bp, synthetic construct
  misc_feature 1..23: note = Description of Artificial Sequence: Synthetic oligonucleotide
  source 1..23: mol_type = other DNA
ctgccatcaaagctaatatttgg

SEQ ID NO: 337 - DNA, 23 bp, synthetic construct
  misc_feature 1..23: note = Description of Artificial Sequence: Synthetic oligonucleotide
  source 1..23: mol_type = other DNA
aaaagttcttactgagcgcttcg

SEQ ID NO: 338 - DNA, 23 bp, synthetic construct
  misc_feature 1..23: note = Description of Artificial Sequence: Synthetic oligonucleotide
  source 1..23: mol_type = other DNA
ctgggatattccgtttacccttg

SEQ ID NO: 339 - DNA, 23 bp, synthetic construct
  misc_feature 1..23: note = Description of Artificial Sequence: Synthetic oligonucleotide
  source 1..23: mol_type = other DNA
tatgaggagactcgaggtgtgct

SEQ ID NO: 340 - DNA, 23 bp, synthetic construct
  misc_feature 1..23: note = Description of Artificial Sequence: Synthetic oligonucleotide
  source 1..23: mol_type = other DNA
agttttcctggattatgcctggc

SEQ ID NO: 341 - DNA, 23 bp, synthetic construct
  misc_feature 1..23: note = Description of Artificial Sequence: Synthetic oligonucleotide
  source 1..23: mol_type = other DNA
gccactccctggccaggctttgg

SEQ ID NO: 342 - DNA, 23 bp, synthetic construct
  misc_feature 1..23: note = Description of Artificial Sequence: Synthetic oligonucleotide
  source 1..23: mol_type = other DNA
tattcatcataggaaacaccaaa

SEQ ID NO: 343 - DNA, 23 bp, synthetic construct
  misc_feature 1..23: note = Description of Artificial Sequence: Synthetic oligonucleotide
  source 1..23: mol_type = other DNA
tgtacatgaagcaactccagtcc

SEQ ID NO: 344 - DNA, 23 bp, synthetic construct
  misc_feature 1..23: note = Description of Artificial Sequence: Synthetic oligonucleotide
  source 1..23: mol_type = other DNA
ccctcccgtcacccctgtttctg

SEQ ID NO: 345 - DNA, 23 bp, synthetic construct
  misc_feature 1..23: note = Description of Artificial Sequence: Synthetic oligonucleotide
  source 1..23: mol_type = other DNA
ttggaatcctggagtgacccctg

SEQ ID NO: 346 - DNA, 23 bp, synthetic construct
  misc_feature 1..23: note = Description of Artificial Sequence: Synthetic oligonucleotide
  source 1..23: mol_type = other DNA
cgtgaacgttcccttagcactct

SEQ ID NO: 347 - DNA, 23 bp, synthetic construct
  misc_feature 1..23: note = Description of Artificial Sequence: Synthetic oligonucleotide
  source 1..23: mol_type = other DNA
gctaaagagggaatgggctttgg

SEQ ID NO: 348 - DNA, 23 bp, synthetic construct
  misc_feature 1..23: note = Description of Artificial Sequence: Synthetic oligonucleotide
  source 1..23: mol_type = other DNA
tcttctgctcggactcaggccct

SEQ ID NO: 349 - DNA, 23 bp, synthetic construct
  misc_feature 1..23: note = Description of Artificial Sequence: Synthetic oligonucleotide
  source 1..23: mol_type = other DNA
gccctcccgtcacccctgtttct

SEQ ID NO: 350 - DNA, 23 bp, synthetic construct
  misc_feature 1..23: note = Description of Artificial Sequence: Synthetic oligonucleotide
  source 1..23: mol_type = other DNA
gacctcccaaacagctacatatt

SEQ ID NO: 351 - DNA, 23 bp, synthetic construct
  misc_feature 1..23: note = Description of Artificial Sequence: Synthetic oligonucleotide
  source 1..23: mol_type = other DNA
ggtgccagaaacaggggtgacgg

SEQ ID NO: 352 - DNA, 23 bp, synthetic construct
  misc_feature 1..23: note = Description of Artificial Sequence: Synthetic oligonucleotide
  source 1..23: mol_type = other DNA
gatggtccatgtctgttactcgc

SEQ ID NO: 353 - DNA, 23 bp, synthetic construct
  misc_feature 1..23: note = Description of Artificial Sequence: Synthetic oligonucleotide
  source 1..23: mol_type = other DNA
tctgtctggtgccatgctgggat

SEQ ID NO: 354 - DNA, 24 bp, synthetic construct
  misc_feature 1..24: note = Description of Artificial Sequence: Synthetic oligonucleotide
  source 1..24: mol_type = other DNA
ctgatggtccatggtctgttactc

SEQ ID NO: 355 - DNA, 23 bp, synthetic construct
  misc_feature 1..23: note = Description of Artificial Sequence: Synthetic oligonucleotide
  source 1..23: mol_type = other DNA
ctgatggtccatggtctgttact

SEQ ID NO: 356 - DNA, 14 bp, synthetic construct
  misc_feature 1..14: note = Description of Artificial Sequence: Synthetic oligonucleotide
  source 1..14: mol_type = other DNA
ctgatggtccatgg

SEQ ID NO: 357 - DNA, 23 bp, synthetic construct
  misc_feature 1..23: note = Description of Artificial Sequence: Synthetic oligonucleotide
  source 1..23: mol_type = other DNA
ctgatggtccatggtctgttact

SEQ ID NO: 358 - DNA, 14 bp, synthetic construct
  misc_feature 1..14: note = Description of Artificial Sequence: Synthetic oligonucleotide
  source 1..14: mol_type = other DNA
ctgatggtccatgg

SEQ ID NO: 359 - protein, 1303 aa, Acidaminococcus sp.
MTQFEGFTNLYQVSKTLRFELIPQGKTLKHIQEQGFIEEDKARNDHYKELKPIIDRIYKTYADQCLQLVQLDWENLSAAIDSYRKEKTEETRNALIEEQATYRNAIHDYFIGRTDNLTDAINKRHAEIYKGLFKAELFNGKVLKQLGTVTTTEHENALLRSFDKFTTYFSGFYENRKNVFSAEDISTAIPHRIVQDNFPKFKENCHIFTRLITAVPSLREHFENVKKAIGIFVSTSIEEVFSFPFYNQLLTQTQIDLYNQLLGGISREAGTEKIKGLNEVLNLAIQKNDETAHIIASLPHRFIPLFKQILSDRNTLSFILEEFKSDEEVIQSFCKYKTLLRNENVLETAEALFNELNSIDLTHIFISHKKLETISSALCDHWDTLRNALYERRISELTGKITKSAKEKVQRSLKHEDINLQEIISAAGKELSEAFKQKTSEILSHAHAALDQPLPTTLKKQEEKEILKSQLDSLLGLYHLLDWFAVDESNEVDPEFSARLTGIKLEMEPSLSFYNKARNYATKKPYSVEKFKLNFQMPTLASGWDVNKEKNNGAILFVKNGLYYLGIMPKQKGRYKALSFEPTEKTSEGFDKMYYDYFPDAAKMIPKCSTQLKAVTAHFQTHTTPILLSNNFIEPLEITKEIYDLNNPEKEPKKFQTAYAKKTGDQKGYREALCKWIDFTRDFLSKYTKTTSIDLSSLRPSSQYKDLGEYYAELNPLLYHISFQRIAEKEIMDAVETGKLYLFQIYNKDFAKGHHGKPNLHTLYWTGLFSPENLAKTSIKLNGQAELFYRPKSRMKRMAHRLGEKMLNKKLKDQKTPIPDTLYQELYDYVNHRLSHDLSDEARALLPNVITKEVSHEIIKDRRFTSDKFFFHVPITLNYQAANSPSKFNQRVNAYLKEHPETPIIGIDRGERNLIYITVIDSTGKILEQRSLNTIQQFDYQKKLDNREKERVAARQAWSVVGTIKDLKQGYLSQVIHEIVDLMIHYQAVVVLENLNFGFKSKRTGIAEKAVYQQFEKMLIDKLNCLVLKDYPAEKVGGVLNPYQLTDQFTSFAKMGTQSGFLFYVPAPYTSKIDPLTGFVDPFVWKTIKNHESRKHFLEGFDFLHYDVKTGDFILHFKMNRNLSFQRGLPGFMPAWDIVFEKNETQFDAKGTPFIAGKRIVPVIENHRFTGRYRDLYPANELIALLEEKGIVFRDGSNILPKLLENDDSHAIDTMVALIRSVLQMRNSNAATGEDYINSPVRDLNGVCFDSRFQNPEWPMDADANGAYHIALKGQLLLNHLKESKDLKLQNGISNQDWLAYIQ

SEQ ID NO: 360 - protein, 1223 aa, unidentified
  REGION 1..1223: note = Description of Unknown: Lachnospiraceae bacterium sequence
MSKLEKFTNCYSLSKTLRFKAIPVGKTQENIDNKRLLVEDEKRAEDYKGVKKLLDRYYLSFINDVLHSIKLKNLNNYISLFRKKTRTEKENKELENLEINLRKEIAKAFKGNEGYKSLFKKDIIETILPEFLDDKDEIALVNSFNGFTTAFTGFFDNRENMFSEEAKSTSIAFRCINENLTRYISNMDIFEKVDAIFDKHEVQEIKEKILNSDYDVEDFFEGEFFNFVLTQEGIDVYNAIIGGFVTESGEKIKGLNEYINLYNQKTKQKLPKFKPLYKQVLSDRESLSFYGEGYTSDEEVLEVFRNTLNKNSEIFSSIKKLEKLFKNFDEYSSAGIFVKNGPAISTISKDIFGEWNVIRDKWNAEYDDIHLKKKAVVTEKYEDDRRKSFKKIGSFSLEQLQEYADADLSVVEKLKEIIIQKVDEIYKVYGSSEKLFDADFVLEKSLKKNDAVVAIMKDLLDSVKSFENYIKAFFGEGKETNRDESFYGDFVLAYDILLKVDHIYDAIRNYVTQKPYSKDKFKLYFQNPQFMGGWDKDKETDYRATILRYGSKYYLAIMDKKYAKCLQKIDKDDVNGNYEKINYKLLPGPNKMLPKVFFSKKWMAYYNPSEDIQKIYKNGTFKKGDMFNLNDCHKLIDFFKDSISRYPKWSNAYDFNFSETEKYKDIAGFYREVEEQGYKVSFESASKKEVDKLVEEGKLYMFQIYNKDFSDKSHGTPNLHTMYFKLLFDENNHGQIRLSGGAELFMRRASLKKEELVVHPANSPIANKNPDNPKKTTTLSYDVYKDKRFSEDQYELHIPIAINKCPKNIFKINTEVRVLLKHDDNPYVIGIDRGERNLLYIVVVDGKGNIVEQYSLNEIINNFNGIRIKTDYHSLLDKKEKERFEARQNWTSIENIKELKAGYISQVVHKICELVEKYDAVIALEDLNSGFKNSRVKVEKQVYQKFEKMLIDKLNYMVDKKSNPCATGGALKGYQITNKFESFKSMSTQNGFIFYIPAWLTSKIDPSTGFVNLLKTKYTSIADSKKFISSFDRIMYVPEEDLFEFALDYKNFSRTDADYIKKWKLYSYGNRIRIFRNPKKNNVFDWEEVCLTSAYKELFNKYGINYQQGDIRALLCEQSDKAFYSSFMALMSLMLQMRNSITGRTDVDFLISPVKNSDGIFYDSRNYEAQENAILPKNADANGAYNIARKVLWAIGQFKKAEDEKLDKVKIAISNKEWLEYAQ

SEQ ID NO: 361 - DNA, 8446 bp, synthetic construct
  misc_feature 1..8446: note = Description of Artificial Sequence: Synthetic polynucleotide
  source 1..8446: mol_type = other DNA
cctgcaggcagctgcgcgctcgctcgctcactgaggccgcccgggcaaagcccgggcgtcgggcgacctttggtcgcccggcctcagtgagcgagcgagcgcgcagagagggagtggccaactccatcactaggggttcctgcggcctctagagagggcctatttcccatgattccttcatatttgcatatacgatacaaggctgttagagagataattggaattaatttgactgtaaacacaaagatattagtacaaaatacgtgacgtagaaagtaataatttcttgggtagtttgcagttttaaaattatgttttaaaatggactatcatatgcttaccgtaacttgaaagtatttcgatttcttggctttatatatcttgtggaaaggacgaaacaccgtaatttctactcttgtagatgggtcttcgagaagacctttttttctattgcatgaagaatctgcttagggttaggcgttttgcgctgcttcgcgatgtacgggccagatatacgcgggtacccgttacataacttacggtaaatggcccgcctggctgaccgcccaacgacccccgcccattgacgtcaatagtaacgccaatagggactttccattgacgtcaatgggtggagtatttacggtaaactgcccacttggcagtacatcaagtgtatcatatgccaagtacgccccctattgacgtcaatgacggtaaatggcccgcctggcattgtgcccagtacatgaccttatgggactttcctacttggcagtacatctacgtattagtcatcgctattaccatggtcgaggtgagccccacgttctgcttcactctccccatctcccccccctccccacccccaattttgtatttatttattttttaattattttgtgcagcgatgggggcggggggggggggggggcgcgcgccaggcggggcggggcggggcgaggggcggggcggggcgaggcggagaggtgcggcggcagccaatcagagcggcgcgctccgaaagtttccttttatggcgaggcggcggcggcggcggccctataaaaagcgaagcgcgcggcgggcgggagtcgctgcgcgctgccttcgccccgtgccccgctccgccgccgcctcgcgccgcccgccccggctctgactgaccgcgttactcccacaggtgagcgggcgggacggcccttctcctccgggctgtaattagctgagcaagaggtaagggtttaagggatggttggttggtggggtattaatgtttaattacctggagcacctgcctgaaatcactttttttcaggttggaccggctagcgtttaaacttaagcttgccaccatggccccaaagaagaagcggaaggtcggtatccacggagtcccagcagccacacagttcgagggctttaccaacctgtatcaggtgagcaagacactgcggtttgagctgatcccacagggcaagaccctgaagcacatccaggagcagggcttcatcgaggaggacaaggcccgcaatgatcactacaaggagctgaagcccatcatcgatcggatctacaagacctatgccgaccagtgcctgcagctggtgcagctggattgggagaacctgagcgccgccatcgactcctatagaaaggagaaaaccgaggagacaaggaacgccctgatcgaggagcaggccacatatcgcaatgccatccacgactacttcatcggccggacagacaacctgaccgatgccatcaataagagacacgccgagatctacaagggcctgttcaaggccgagctgtttaatggcaaggtgctgaagcagctgggcaccgtgaccacaaccgagcacgagaacgccctgctgcggagcttcgacaagtttacaacctacttctccggcttttatgagaacaggaagaacgtgttcagcgccgaggatatcagcacagccatcccacaccgcatcgtgcaggacaacttccccaagtttaaggagaattgtcacatcttcacacgcctgatcaccgccgtgcccagcctgcgggagcactttgagaacgtgaagaaggccatcggcatcttcgtgagcacctccatcgaggaggtgttttccttccctttttataaccagctgctgacacagacccagatcgacctgtataaccagctgctgggaggaatctctcgggaggcaggcaccgagaagatcaagggcctgaacgaggtgctgaatctggccatccagaagaatgatgagacagcccacatcatcgcctccctgccacacagattcatccccctgtttaagcagatcctgtccgataggaacaccctgtctttcatcctggaggagtttaagagcgacgaggaagtgatccagtccttctgcaagtacaagacactgctgagaaacgagaacgtgctggagacagccgaggccctgtttaacgagctgaacagcatcgacctgacacacatcttcatcagccacaagaagctggagacaatcagcagcgccctgtgcgaccactgggatacactgaggaatgccctgtatgagcggagaatctccgagctgacaggcaagatcaccaagtctgccaaggagaaggtgcagcgcagcctgaagcacgaggatatcaacctgcaggagatcatctctgccgcaggcaaggagctgagcgaggccttcaagcagaaaaccagcgagatcctgtcccacgcacacgccgccctggatcagccactgcctacaaccctgaagaagcaggaggagaaggagatcctgaagtctcagctggacagcctgctgggcctgtaccacctgctggactggtttgccgtggatgagtccaacgaggtggaccccgagttctctgcccggctgaccggcatcaagctggagatggagccttctctgagcttctacaacaaggccagaaattatgccaccaagaagccctactccgtggagaagttcaagctgaactttcagatgcctacactggcccggggctgggacgtgaataaggagaagaacaatggcgccatcctgtttgtgaagaacggcctgtactatctgggcatcatgccaaagcagaagggcaggtataaggccctcagcttcgagcccacagagaaaaccagcgagggctttgataagatgtactatgactactttccggatgccgccaagatgatcccacggtgcagcacccagctgaaggcggtgaccgcccactttcagacccacacaacccccatcctgctgtccaacaatttcatcgagcctctggagatcacaaaggagatctacgacctgaacaatcctgagaaggagccaaagaagtttcagacagcgtacgccaagaaaaccggcgaccagaagggctacagagaggccctgtgcaagtggatcgacttcacaagggattttctgtccaagtataccaagacaacctctatcgatctgtctagcctgcggccatcctctcagtataaggacctgggcgagtactatgccgagctgaatcccctgctgtaccacatcagcttccagagaatcgccgagaaggagatcatggatgccgtggagacaggcaagctgtacctgttccagatctataacaaggactttgccaagggccaccacggcaagcctaatctgcacacactgtattggaccggtctgttttctccagagaacctggccaagacaagcatcaagctgaatggccaggccgagctgttctaccgccctaagtccaggatgaagaggatggcacaccggctgggagagaagatgctgaacaagaagctgaaggatcagaaaaccccaatccccgacaccctgtaccaggagctgtacgactatgtgaatcacagactgtcccacgacctgtctgatgaggccagggccctgctgcccaacgtgatcaccaaggaggtgtctcacgagatcatcaaggataggcgctttaccagcgacaagttctttttccacgtgcctatcacactgaactatcaggccgccaattccccatctaagttcaaccagagggtgaatgcctacctgaaggagcaccccgagacacctatcatcggcatcgatcggggcgagagaaacctgatctatatcacagtgatcgactccaccggcaagatcctggagcagcggagcctgaacaccatccagcagtttgattaccagaagaagctggacaacagggagaaggagagggtggcagcaaggcaggcctggtctgtggtgggcacaatcaaggatctgaagcagggctatctgagccaggtcatccacgagatcgtggacctgatgatccactaccaggccgtggtggtgctggagaacctgaatttcggctttaagagcaagaggaccggcatcgccgagaaggccgtgtaccagcagttcgagaagatgctgatcgataagctgaattgcctggtgctgaaggactatccagcagagaaagtgggaggcgtgctgaacccataccagctgacagaccagttcacctcctttgccaagatgggcacccagtctggcttcctgttttacgtgcctgccccatatacatctaagatcgatcccctgaccggcttcgtggaccccttcgtgtggaaaaccatcaagaatcacgagagccgcaagcacttcctggagggcttcgactttctgcactacgacgtgaaaaccggcgacttcatcctgcactttaagatgaacagaaatctgtccttccagaggggcctgcccggctttatgcctgcatgggatatcgtgttcgagaagaacgagacacagtttgacgccaagggcacccctttcatcgccggcaagagaatcgtgccagtgatcgagaatcacagattcaccggcagataccgggacctgtatcctgccaacgagctgatcgccctgctggaggagaagggcatcgtgttcagggatggctccaacatcctgccaaagctgctggagaatgacgattctcacgccatcgacaccatggtggccctgatccgcagcgtgctgcagatgcggaactccaatgccgccacaggcgaggactatatcaacagccccgtgcgcgatctgaatggcgtgtgcttcgactcccggtttcagaacccagagtggcccatggacgccgatgccaatggcgcctaccacatcgccctgaagggccagctgctgctgaatcacctgaaggagagcaaggatctgaagctgcagaacggcatctccaatcaggactggctggcctacatccaggagctgcgcaacaaaaggccggcggccacgaaaaaggccggccaggcaaaaaagaaaaagggatcctacccatacgatgttccagattacgcttatccctacgacgtgcctgattatgcatacccatatgatgtccccgactatgcctaagaattcctagagctcgctgatcagcctcgactgtgccttctagttgccagccatctgttgtttgcccctcccccgtgccttccttgaccctggaaggtgccactcccactgtcctttcctaataaaatgaggaaattgcatcgcattgtctgagtaggtgtcattctattctggggggtggggtggggcaggacagcaagggggaggattgggaagagaatagcaggcatgctggggagcggccgcaggaacccctagtgatggagttggccactccctctctgcgcgctcgctcgctcactgaggccgggcgaccaaaggtcgcccgacgcccgggctttgcccgggcggcctcagtgagcgagcgagcgcgcagctgcctgcaggggcgcctgatgcggtattttctccttacgcatctgtgcggtatttcacaccgcatacgtcaaagcaaccatagtacgcgccctgtagcggcgcattaagcgcggcgggtgtggtggttacgcgcagcgtgaccgctacacttgccagcgccctagcgcccgctcctttcgctttcttcccttcctttctcgccacgttcgccggctttccccgtcaagctctaaatcgggggctccctttagggttccgatttagtgctttacggcacctcgaccccaaaaaacttgatttgggtgatggttcacgtagtgggccatcgccctgatagacggtttttcgccctttgacgttggagtccacgttctttaatagtggactcttgttccaaactggaacaacactcaaccctatctcgggctattcttttgatttataagggattttgccgatttcggcctattggttaaaaaatgagctgatttaacaaaaatttaacgcgaattttaacaaaatattaacgtttacaattttatggtgcactctcagtacaatctgctctgatgccgcatagttaagccagccccgacacccgccaacacccgctgacgcgccctgacgggcttgtctgctcccggcatccgcttacagacaagctgtgaccgtctccgggagctgcatgtgtcagaggttttcaccgtcatcaccgaaacgcgcgagacgaaagggcctcgtgatacgcctatttttataggttaatgtcatgataataatggtttcttagacgtcaggtggcacttttcggggaaatgtgcgcggaacccctatttgtttatttttctaaatacattcaaatatgtatccgctcatgagacaataaccctgataaatgcttcaataatattgaaaaaggaagagtatgagtattcaacatttccgtgtcgcccttattcccttttttgcggcattttgccttcctgtttttgctcacccagaaacgctggtgaaagtaaaagatgctgaagatcagttgggtgcacgagtgggttacatcgaactggatctcaacagcggtaagatccttgagagttttcgccccgaagaacgttttccaatgatgagcacttttaaagttctgctatgtggcgcggtattatcccgtattgacgccgggcaagagcaactcggtcgccgcatacactattctcagaatgacttggttgagtactcaccagtcacagaaaagcatcttacggatggcatgacagtaagagaattatgcagtgctgccataaccatgagtgataacactgcggccaacttacttctgacaacgatcggaggaccgaaggagctaaccgcttttttgcacaacatgggggatcatgtaactcgccttgatcgttgggaaccggagctgaatgaagccataccaaacgacgagcgtgacaccacgatgcctgtagcaatggcaacaacgttgcgcaaactattaactggcgaactacttactctagcttcccggcaacaattaatagactggatggaggcggataaagttgcaggaccacttctgcgctcggcccttccggctggctggtttattgctgataaatctggagccggtgagcgtggaagccgcggtatcattgcagcactggggccagatggtaagccctcccgtatcgtagttatctacacgacggggagtcaggcaactatggatgaacgaaatagacagatcgctgagataggtgcctcactgattaagcattggtaactgtcagaccaagtttactcatatatactttagattgatttaaaacttcatttttaatttaaaaggatctaggtgaagatcctttttgataatctcatgaccaaaatcccttaacgtgagttttcgttccactgagcgtcagaccccgtagaaaagatcaaaggatcttcttgagatcctttttttctgcgcgtaatctgctgcttgcaaacaaaaaaaccaccgctaccagcggtggtttgtttgccggatcaagagctaccaactctttttccgaaggtaactggcttcagcagagcgcagataccaaatactgtccttctagtgtagccgtagttaggccaccacttcaagaactctgtagcaccgcctacatacctcgctctgctaatcctgttaccagtggctgctgccagtggcgataagtcgtgtcttaccgggttggactcaagacgatagttaccggataaggcgcagcggtcgggctgaacggggggttcgtgcacacagcccagcttggagcgaacgacctacaccgaactgagatacctacagcgtgagctatgagaaagcgccacgcttcccgaagggagaaaggcggacaggtatccggtaagcggcagggtcggaacaggagagcgcacgagggagcttccagggggaaacgcctggtatctttatagtcctgtcgggtttcgccacctctgacttgagcgtcgatttttgtgatgctcgtcaggggggcggagcctatggaaaaacgccagcaacgcggcctttttacggttcctggccttttgctggccttttgctcacatgt

SEQ ID NO: 362 - protein, 1351 aa, synthetic construct
  REGION 1..1351: note = Description of Artificial Sequence: Synthetic polypeptide
TQFEGFTNLYQVSKTLRFELIPQGKTLKHIQEQGFIEEDKARNDHYKELKPIIDRIYKTYADQCLQLVQLDWENLSAAIDSYRKEKTEETRNALIEEQATYRNAIHDYFIGRTDNLTDAINKRHAEIYKGLFKAELFNGKVLKQLGTVTTTEHENALLRSFDKFTTYFSGFYENRKNVFSAEDISTAIPHRIVQDNFPKFKENCHIFTRLITAVPSLREHFENVKKAIGIFVSTSIEEVFSFPFYNQLLTQTQIDLYNQLLGGISREAGTEKIKGLNEVLNLAIQKNDETAHIIASLPHRFIPLFKQILSDRNTLSFILEEFKSDEEVIQSFCKYKTLLRNENVLETAEALFNELNSIDLTHIFISHKKLETISSALCDHWDTLRNALYERRISELTGKITKSAKEKVQRSLKHEDINLQEIISAAGKELSEAFKQKTSEILSHAHAALDQPLPTTLKKQEEKEILKSQLDSLLGLYHLLDWFAVDESNEVDPEFSARLTGIKLEMEPSLSFYNKARNYATKKPYSVEKFKLNFQMPTLARGWDVNKEKNNGAILFVKNGLYYLGIMPKQKGRYKALSFEPTEKTSEGFDKMYYDYFPDAAKMIPRCSTQLKAVTAHFQTHTTPILLSNNFIEPLEITKEIYDLNNPEKEPKKFQTAYAKKTGDQKGYREALCKWIDFTRDFLSKYTKTTSIDLSSLRPSSQYKDLGEYYAELNPLLYHISFQRIAEKEIMDAVETGKLYLFQIYNKDFAKGHHGKPNLHTLYWTGLFSPENLAKTSIKLNGQAELFYRPKSRMKRMAHRLGEKMLNKKLKDQKTPIPDTLYQELYDYVNHRLSHDLSDEARALLPNVITKEVSHEIIKDRRFTSDKFFFHVPITLNYQAANSPSKFNQRVNAYLKEHPETPIIGIDRGERNLIYITVIDSTGKILEQRSLNTIQQFDYQKKLDNREKERVAARQAWSVVGTIKDLKQGYLSQVIHEIVDLMIHYQAVVVLENLNFGFKSKRTGIAEKAVYQQFEKMLIDKLNCLVLKDYPAEKVGGVLNPYQLTDQFTSFAKMGTQSGFLFYVPAPYTSKIDPLTGFVDPFVWKTIKNHESRKHFLEGFDFLHYDVKTGDFILHFKMNRNLSFQRGLPGFMPAWDIVFEKNETQFDAKGTPFIAGKRIVPVIENHRFTGRYRDLYPANELIALLEEKGIVFRDGSNILPKLLENDDSHAIDTMVALIRSVLQMRNSNAATGEDYINSPVRDLNGVCFDSRFQNPEWPMDADANGAYHIALKGQLLLNHLKESKDLKLQNGISNQDWLAYIQELRNKRPAATKKAGQAKKKKGSYPYDVPDYAYPYDVPDYAYPYDVPDYA

SEQ ID NO: 363 - DNA, 9464 bp, synthetic construct
  misc_feature 1..9464: note = Description of Artificial Sequence: Synthetic polynucleotide
  source 1..9464: mol_type = other DNA
gacggatcgggagatctcccgatcccctatggtgcactctcagtacaatctgctctgatgccgcatagttaagccagtatctgctccctgcttgtgtgttggaggtcgctgagtagtgcgcgagcaaaatttaagctacaacaaggcaaggcttgaccgacaattgcatgaagaatctgcttagggttaggcgttttgcgctgcttcgcgatgtacgggccagatatacgcgttgacattgattattgactagttattaatagtaatcaattacggggtcattagttcatagcccatatatggagttccgcgttacataacttacggtaaatggcccgcctggctgaccgcccaacgacccccgcccattgacgtcaataatgacgtatgttcccatagtaacgccaatagggactttccattgacgtcaatgggtggagtatttacggtaaactgcccacttggcagtacatcaagtgtatcatatgccaagtacgccccctattgacgtcaatgacggtaaatggcccgcctggcattatgcccagtacatgaccttatgggactttcctacttggcagtacatctacgtattagtcatcgctattaccatggtgatgcggttttggcagtacatcaatgggcgtggatagcggtttgactcacggggatttccaagtctccaccccattgacgtcaatgggagtttgttttggcaccaaaatcaacgggactttccaaaatgtcgtaacaactccgccccattgacgcaaatgggcggtaggcgtgtacggtgggaggtctatataagcagagctctctggctaactagagaacccactgcttactggcttatcgaaattaatacgactcactatagggagacccaagctggctagcgtttaaacttaagcttggtaccgccaccatgacacagttcgagggctttaccaacctgtatcaggtgagcaagacactgcggtttgagctgatcccacagggcaagaccctgaagcacatccaggagcagggcttcatcgaggaggacaaggcccgcaatgatcactacaaggagctgaagcccatcatcgatcggatctacaagacctatgccgaccagtgcctgcagctggtgcagctggattgggagaacctgagcgccgccatcgactcctatagaaaggagaaaaccgaggagacaaggaacgccctgatcgaggagcaggccacatatcgcaatgccatccacgactacttcatcggccggacagacaacctgaccgatgccatcaataagagacacgccgagatctacaagggcctgttcaaggccgagctgtttaatggcaaggtgctgaagcagctgggcaccgtgaccacaaccgagcacgagaacgccctgctgcggagcttcgacaagtttacaacctacttctccggcttttatgagaacaggaagaacgtgttcagcgccgaggatatcagcacagccatcccacaccgcatcgtgcaggacaacttccccaagtttaaggagaattgtcacatcttcacacgcctgatcaccgccgtgcccagcctgcgggagcactttgagaacgtgaagaaggccatcggcatcttcgtgagcacctccatcgaggaggtgttttccttccctttttataaccagctgctgacacagacccagatcgacctgtataaccagctgctgggaggaatctctcgggaggcaggcaccgagaagatcaagggcctgaacgaggtgctgaatctggccatccagaagaatgatgagacagcccacatcatcgcctccctgccacacagattcatccccctgtttaagcagatcctgtccgataggaacaccctgtctttcatcctggaggagtttaagagcgacgaggaagtgatccagtccttctgcaagtacaagacactgctgagaaacgagaacgtgctggagacagccgaggccctgtttaacgagctgaacagcatcgacctgacacacatcttcatcagccacaagaagctggagacaatcagcagcgccctgtgcgaccactgggatacactgaggaatgccctgtatgagcggagaatctccgagctgacaggcaagatcaccaagtctgccaaggagaaggtgcagcgcagcctgaagcacgaggatatcaacctgcaggagatcatctctgccgcaggcaaggagctgagcgaggccttcaagcagaaaaccagcgagatcctgtcccacgcacacgccgccctggatcagccactgcctacaaccctgaagaagcaggaggagaaggagatcctgaagtctcagctggacagcctgctgggcctgtaccacctgctggactggtttgccgtggatgagtccaacgaggtggaccccgagttctctgcccggctgaccggcatcaagctggagatggagccgtctctgagcttctacaacaaggccagaaattatgccaccaagaagccctactccgtggagaagttcaagctgaactttcagatgcctacactggcccggggctgggacgtgaataaggagaagaacaatggcgccatcctgtttgtgaagaacggcctgtactatctgggcatcatgccaaagcagaagggcaggtataaggccctcagcttcgagcccacagagaaaaccagcgagggctttgataagatgtactatgactactttccggatgccgccaagatgatcccacggtgcagcacccagctgaaggcggtgaccgcccactttcagacccacacaacccccatcctgctgtccaacaatttcatcgagcctctggagatcacaaaggagatctacgacctgaacaatcctgagaaggagccaaagaagtttcagacagcgtacgccaagaaaaccggcgaccagaagggctacagagaggccctgtgcaagtggatcgacttcacaagggattttctgtccaagtataccaagacaacctctatcgatctgtctagcctgcggccatcctctcagtataaggacctgggcgagtactatgccgagctgaatcccctgctgtaccacatcagcttccagagaatcgccgagaaggagatcatggatgccgtggagacaggcaagctgtacctgttccagatctataacaaggactttgccaagggccaccacggcaagcctaatctgcacacactgtattggaccggtctgttttctccagagaacctggccaagacaagcatcaagctgaatggccaggccgagctgttctaccgccctaagtccaggatgaagaggatggcacaccggctgggagagaagatgctgaacaagaagctgaaggatcagaaaaccccaatccccgacaccctgtaccaggagctgtacgactatgtgaatcacagactgtcccacgacctgtctgatgaggccagggccctgctgcccaacgtgatcaccaaggaggtgtctcacgagatcatcaaggataggcgctttaccagcgacaagttctttttccacgtgcctatcacactgaactatcaggccgccaattccccatctaagttcaaccagagggtgaatgcctacctgaaggagcaccccgagacacctatcatcggcatcgatcggggcgagagaaacctgatctatatcacagtgatcgactccaccggcaagatcctggagcagcggagcctgaacaccatccagcagtttgattaccagaagaagctggacaacagggagaaggagagggtggcagcaaggcaggcctggtctgtggtgggcacaatcaaggatctgaagcagggctatctgagccaggtcatccacgagatcgtggacctgatgatccactaccaggccgtggtggtgctggagaacctgaatttcggctttaagagcaagaggaccggcatcgccgagaaggccgtgtaccagcagttcgagaagatgctgatcgataagctgaattgcctggtgctgaaggactatccagcagagaaagtgggaggcgtgctgaacccataccagctgacagaccagttcacctcctttgccaagatgggcacccagtctggcttcctgttttacgtgcctgccccatatacatctaagatcgatcccctgaccggcttcgtggaccccttcgtgtggaaaaccatcaagaatcacgagagccgcaagcacttcctggagggcttcgactttctgcactacgacgtgaaaaccggcgacttcatcctgcactttaagatgaacagaaatctgtccttccagaggggcctgcccggctttatgcctgcatgggatatcgtgttcgagaagaacgagacacagtttgacgccaagggcacccctttcatcgccggcaagagaatcgtgccagtgatcgagaatcacagattcaccggcagataccgggacctgtatcctgccaacgagctgatcgccctgctggaggagaagggcatcgtgttcagggatggctccaacatcctgccaaagctgctggagaatgacgattctcacgccatcgacaccatggtggccctgatccgcagcgtgctgcagatgcggaactccaatgccgccacaggcgaggactatatcaacagccccgtgcgcgatctgaatggcgtgtgcttcgactcccggtttcagaacccagagtggcccatggacgccgatgccaatggcgcctaccacatcgccctgaagggccagctgctgctgaatcacctgaaggagagcaaggatctgaagctgcagaacggcatctccaatcaggactggctggcctacatccaggagctgcgcaacaaaaggccggcggccacgaaaaaggccggccaggcaaaaaagaaaaagggatcctacccatacgatgttccagattacgcttatccctacgacgtgcctgattatgcatacccatatgatgtccccgactatgcctaagaattctgcagatatccagcacagtggcggccgctcgagtctagagggcccgtttaaacccgctgatcagcctcgactgtgccttctagttgccagccatctgttgtttgcccctcccccgtgccttccttgaccctggaaggtgccactcccactgtcctttcctaataaaatgaggaaattgcatcgcattgtctgagtaggtgtcattctattctggggggtggggtggggcaggacagcaagggggaggattgggaagacaatagcaggcatgctggggatgcggtgggctctatggcttctgaggcggaaagaaccagctggggctctagggggtatccccacgcgccctgtagcggcgcattaagcgcggcgggtgtggtggttacgcgcagcgtgaccgctacacttgccagcgccctagcgcccgctcctttcgctttcttcccttcctttctcgccacgttcgccggctttccccgtcaagctctaaatcgggggctccctttagggttccgatttagtgctttacggcacctcgaccccaaaaaacttgattagggtgatggttcacgtagtgggccatcgccctgatagacggtttttcgccctttgacgttggagtccacgttctttaatagtggactcttgttccaaactggaacaacactcaaccctatctcggtctattcttttgatttataagggattttgccgatttcggcctattggttaaaaaatgagctgatttaacaaaaatttaacgcgaattaattctgtggaatgtgtgtcagttagggtgtggaaagtccccaggctccccagcaggcagaagtatgcaaagcatgcatctcaattagtcagcaaccaggtgtggaaagtccccaggctccccagcaggcagaagtatgcaaagcatgcatctcaattagtcagcaaccatagtcccgcccctaactccgcccatcccgcccctaactccgcccagttccgcccattctccgccccatggctgactaattttttttatttatgcagaggccgaggccgcctctgcctctgagctattccagaagtagtgaggaggcttttttggaggcctaggcttttgcaaaaagctcccgggagcttgtatatccattttcggatctgatcaagagacaggatgaggatcgtttcgcatgattgaacaagatggattgcacgcaggttctccggccgcttgggtggagaggctattcggctatgactgggcacaacagacaatcggctgctctgatgccgccgtgttccggctgtcagcgcaggggcgcccggttctttttgtcaagaccgacctgtccggtgccctgaatgaactgcaggacgaggcagcgcggctatcgtggctggccacgacgggcgttccttgcgcagctgtgctcgacgttgtcactgaagcgggaagggactggctgctattgggcgaagtgccggggcaggatctcctgtcatctcaccttgctcctgccgagaaagtatccatcatggctgatgcaatgcggcggctgcatacgcttgatccggctacctgcccattcgaccaccaagcgaaacatcgcatcgagcgagcacgtactcggatggaagccggtcttgtcgatcaggatgatctggacgaagagcatcaggggctcgcgccagccgaactgttcgccaggctcaaggcgcgcatgcccgacggcgaggatctcgtcgtgacccatggcgatgcctgcttgccgaatatcatggtggaaaatggccgcttttctggattcatcgactgtggccggctgggtgtggcggaccgctatcaggacatagcgttggctacccgtgatattgctgaagagcttggcggcgaatgggctgaccgcttcctcgtgctttacggtatcgccgctcccgattcgcagcgcatcgccttctatcgccttcttgacgagttcttctgagcgggactctggggttcgaaatgaccgaccaagcgacgcccaacctgccatcacgagatttcgattccaccgccgccttctatgaaaggttgggcttcggaatcgttttccgggacgccggctggatgatcctccagcgcggggatctcatgctggagttcttcgcccaccccaacttgtttattgcagcttataatggttacaaataaagcaatagcatcacaaatttcacaaataaagcatttttttcactgcattctagttgtggtttgtccaaactcatcaatgtatcttatcatgtctgtataccgtcgacctctagctagagcttggcgtaatcatggtcatagctgtttcctgtgtgaaattgttatccgctcacaattccacacaacatacgagccggaagcataaagtgtaaagcctggggtgcctaatgagtgagctaactcacattaattgcgttgcgctcactgcccgctttccagtcgggaaacctgtcgtgccagctgcattaatgaatcggccaacgcgcggggagaggcggtttgcgtattgggcgctcttccgcttcctcgctcactgactcgctgcgctcggtcgttcggctgcggcgagcggtatcagctcactcaaaggcggtaatacggttatccacagaatcaggggataacgcaggaaagaacatgtgagcaaaaggccagcaaaaggccaggaaccgtaaaaaggccgcgttgctggcgtttttccataggctccgcccccctgacgagcatcacaaaaatcgacgctcaagtcagaggtggcgaaacccgacaggactataaagataccaggcgtttccccctggaagctccctcgtgcgctctcctgttccgaccctgccgcttaccggatacctgtccgcctttctcccttcgggaagcgtggcgctttctcatagctcacgctgtaggtatctcagttcggtgtaggtcgttcgctccaagctgggctgtgtgcacgaaccccccgttcagcccgaccgctgcgccttatccggtaactatcgtcttgagtccaacccggtaagacacgacttatcgccactggcagcagccactggtaacaggattagcagagcgaggtatgtaggcggtgctacagagttcttgaagtggtggcctaactacggctacactagaagaacagtatttggtatctgcgctctgctgaagccagttaccttcggaaaaagagttggtagctcttgatccggcaaacaaaccaccgctggtagcggtttttttgtttgcaagcagcagattacgcgcagaaaaaaaggatctcaagaagatcctttgatcttttctacggggtctgacgctcagtggaacgaaaactcacgttaagggattttggtcatgagattatcaaaaaggatcttcacctagatccttttaaattaaaaatgaagttttaaatcaatctaaagtatatatgagtaaacttggtctgacagttaccaatgcttaatcagtgaggcacctatctcagcgatctgtctatttcgttcatccatagttgcctgactccccgtcgtgtagataactacgatacgggagggcttaccatctggccccagtgctgcaatgataccgcgagacccacgctcaccggctccagatttatcagcaataaaccagccagccggaagggccgagcgcagaagtggtcctgcaactttatccgcctccatccagtctattaattgttgccgggaagctagagtaagtagttcgccagttaatagtttgcgcaacgttgttgccattgctacaggcatcgtggtgtcacgctcgtcgtttggtatggcttcattcagctccggttcccaacgatcaaggcgagttacatgatcccccatgttgtgcaaaaaagcggttagctccttcggtcctccgatcgttgtcagaagtaagttggccgcagtgttatcactcatggttatggcagcactgcataattctcttactgtcatgccatccgtaagatgcttttctgtgactggtgagtactcaaccaagtcattctgagaatagtgtatgcggcgaccgagttgctcttgcccggcgtcaatacgggataataccgcgccacatagcagaactttaaaagtgctcatcattggaaaacgttcttcggggcgaaaactctcaaggatcttaccgctgttgagatccagttcgatgtaacccactcgtgcacccaactgatcttcagcatcttttactttcaccagcgtttctgggtgagcaaaaacaggaaggcaaaatgccgcaaaaaagggaataagggcgacacggaaatgttgaatactcatactcttcctttttcaatattattgaagcatttatcagggttattgtctcatgagcggatacatatttgaatgtatttagaaaaataaacaaataggggttccgcgcacatttccccgaaaagtgccacctgacgtc

SEQ ID NO: 364 - protein, 1352 aa, synthetic construct
  REGION 1..1352: note = Description of Artificial Sequence: Synthetic polypeptide
MTQFEGFTNLYQVSKTLRFELIPQGKTLKHIQEQGFIEEDKARNDHYKELKPIIDRIYKTYADQCLQLVQLDWENLSAAIDSYRKEKTEETRNALIEEQATYRNAIHDYFIGRTDNLTDAINKRHAEIYKGLFKAELFNGKVLKQLGTVTTTEHENALLRSFDKFTTYFSGFYENRKNVFSAEDISTAIPHRIVQDNFPKFKENCHIFTRLITAVPSLREHFENVKKAIGIFVSTSIEEVFSFPFYNQLLTQTQIDLYNQLLGGISREAGTEKIKGLNEVLNLAIQKNDETAHIIASLPHRFIPLFKQILSDRNTLSFILEEFKSDEEVIQSFCKYKTLLRNENVLETAEALFNELNSIDLTHIFISHKKLETISSALCDHWDTLRNALYERRISELTGKITKSAKEKVQRSLKHEDINLQEIISAAGKELSEAFKQKTSEILSHAHAALDQPLPTTLKKQEEKEILKSQLDSLLGLYHLLDWFAVDESNEVDPEFSARLTGIKLEMEPSLSFYNKARNYATKKPYSVEKFKLNFQMPTLARGWDVNKEKNNGAILFVKNGLYYLGIMPKQKGRYKALSFEPTEKTSEGFDKMYYDYFPDAAKMIPRCSTQLKAVTAHFQTHTTPILLSNNFIEPLEITKEIYDLNNPEKEPKKFQTAYAKKTGDQKGYREALCKWIDFTRDFLSKYTKTTSIDLSSLRPSSQYKDLGEYYAELNPLLYHISFQRIAEKEIMDAVETGKLYLFQIYNKDFAKGHHGKPNLHTLYWTGLFSPENLAKTSIKLNGQAELFYRPKSRMKRMAHRLGEKMLNKKLKDQKTPIPDTLYQELYDYVNHRLSHDLSDEARALLPNVITKEVSHEIIKDRRFTSDKFFFHVPITLNYQAANSPSKFNQRVNAYLKEHPETPIIGIDRGERNLIYITVIDSTGKILEQRSLNTIQQFDYQKKLDNREKERVAARQAWSVVGTIKDLKQGYLSQVIHEIVDLMIHYQAVVVLENLNFGFKSKRTGIAEKAVYQQFEKMLIDKLNCLVLKDYPAEKVGGVLNPYQLTDQFTSFAKMGTQSGFLFYVPAPYTSKIDPLTGFVDPFVWKTIKNHESRKHFLEGFDFLHYDVKTGDFILHFKMNRNLSFQRGLPGFMPAWDIVFEKNETQFDAKGTPFIAGKRIVPVIENHRFTGRYRDLYPANELIALLEEKGIVFRDGSNILPKLLENDDSHAIDTMVALIRSVLQMRNSNAATGEDYINSPVRDLNGVCFDSRFQNPEWPMDADANGAYHIALKGQLLLNHLKESKDLKLQNGISNQDWLAYIQELRNKRPAATKKAGQAKKKKGSYPYDVPDYAYPYDVPDYAYPYDVPDYA

SEQ ID NO: 365 - DNA, 31 bp, synthetic construct
  misc_feature 1..31: note = Description of Artificial Sequence: Synthetic oligonucleotide
  misc_difference 1..8: note = a, c, t, g, unknown or other
  source 1..31: mol_type = other DNA
nnnnnnnngagaagtcatttaataaggccac

SEQ ID NO: 366 - RNA, 23 nt, synthetic construct
  misc_feature 1..23: note = Description of Artificial Sequence: Synthetic oligonucleotide
  source 1..23: mol_type = other RNA
gagaagtcatttaataaggccac

SEQ ID NO: 367 - DNA, 27 bp, synthetic construct
  misc_feature 1..27: note = Description of Artificial Sequence: Synthetic oligonucleotide
  misc_difference 1..8: note = a, c, t, g, unknown or other
  source 1..27: mol_type = other DNA
nnnnnnnngagaagtcatttaataagg

SEQ ID NO: 368 - DNA, 31 bp, synthetic construct
  misc_feature 1..31: note = Description of Artificial Sequence: Synthetic oligonucleotide
  misc_difference 24..31: note = a, c, t, g, unknown or other
  source 1..31: mol_type = other DNA
gtggccttattaaatgacttctcnnnnnnnn

SEQ ID NO: 369 - DNA, 27 bp, synthetic construct
  misc_feature 1..27: note = Description of Artificial Sequence: Synthetic oligonucleotide
  source 1..27: mol_type = other DNA
tttgctaggaatattgaagggggcagg

SEQ ID NO: 370 - DNA, 27 bp, synthetic construct
  misc_feature 1..27: note = Description of Artificial Sequence: Synthetic oligonucleotide
  source 1..27: mol_type = other DNA
catagcaggtattttgaagggggcagg

SEQ ID NO: 371 - DNA, 27 bp, synthetic construct
  misc_feature 1..27: note = Description of Artificial Sequence: Synthetic oligonucleotide
  source 1..27: mol_type = other DNA
tttggtgctcaatgaaaggagataagg

SEQ ID NO: 372 - DNA, 27 bp, synthetic construct
  misc_feature 1..27: note = Description of Artificial Sequence: Synthetic oligonucleotide
  source 1..27: mol_type = other DNA
tttgaagaaatattacaacatataaaa

SEQ ID NO: 373 - DNA, 28 bp, synthetic construct
  misc_feature 1..28: note = Description of Artificial Sequence: Synthetic oligonucleotide
  source 1..28: mol_type = other DNA
cataaacaaatatcactaatatataaaa

SEQ ID NO: 374 - DNA, 27 bp, synthetic construct
  misc_feature 1..27: note = Description of Artificial Sequence: Synthetic oligonucleotide
  source 1..27: mol_type = other DNA
agagaagcagtatcacaacatattaaa

SEQ ID NO: 375 - DNA, 28 bp, synthetic construct
  misc_feature 1..28: note = Description of Artificial Sequence: Synthetic oligonucleotide
  source 1..28: mol_type = other DNA
taaagagaaatatttcatcatgataaaa

SEQ ID NO: 376 - DNA, 28 bp, synthetic construct
  misc_feature 1..28: note = Description of Artificial Sequence: Synthetic oligonucleotide
  source 1..28: mol_type = other DNA
aacaaagaaatattagaaaataattaaa

SEQ ID NO: 377 - DNA, 27 bp, synthetic construct
  misc_feature 1..27: note = Description of Artificial Sequence: Synthetic oligonucleotide
  source 1..27: mol_type = other DNA
tttgtcctccggttctggaaccacacc

SEQ ID NO: 378 - DNA, 27 bp, synthetic construct
  misc_feature 1..27: note = Description of Artificial Sequence: Synthetic oligonucleotide
  source 1..27: mol_type = other DNA
ttcatcctccggttctggaaccagatt

SEQ ID NO: 379 - DNA, 27 bp, synthetic construct
  misc_feature 1..27: note = Description of Artificial Sequence: Synthetic oligonucleotide
  source 1..27: mol_type = other DNA
ttcatcctccggttctggaaccagatc

SEQ ID NO: 380 - DNA, 27 bp, synthetic construct
  misc_feature 1..27: note = Description of Artificial Sequence: Synthetic oligonucleotide
  source 1..27: mol_type = other DNA
ttcatcctccggttctgaaaccacact

SEQ ID NO: 381 - DNA, 27 bp, synthetic construct
  misc_feature 1..27: note = Description of Artificial Sequence: Synthetic oligonucleotide
  source 1..27: mol_type = other DNA
ttcatcctccggttctgaaaccagatc

SEQ ID NO: 382 - DNA, 27 bp, synthetic construct
  misc_feature 1..27: note = Description of Artificial Sequence: Synthetic oligonucleotide
  source 1..27: mol_type = other DNA
ttcatcctctggttctggaaccaggtc

SEQ ID NO: 383 - DNA, 27 bp, synthetic construct
  misc_feature 1..27: note = Description of Artificial Sequence: Synthetic oligonucleotide
  source 1..27: mol_type = other DNA
ttcatccttcggttctggaaccagatc

SEQ ID NO: 384 - DNA, 27 bp, synthetic construct
  misc_feature 1..27: note = Description of Artificial Sequence: Synthetic oligonucleotide
  source 1..27: mol_type = other DNA
tttggggtgatcagacccaacagcagg

SEQ ID NO: 385 - DNA, 27 bp, synthetic construct
  misc_feature 1..27: note = Description of Artificial Sequence: Synthetic oligonucleotide
  source 1..27: mol_type = other DNA
tttggggtgatcagacccaacaccagg

SEQ ID NO: 386 - DNA, 27 bp, synthetic construct
  misc_feature 1..27: note = Description of Artificial Sequence: Synthetic oligonucleotide
  source 1..27: mol_type = other DNA
tttggggtgatcagacccaaccccagg

SEQ ID NO: 387 - DNA, 27 bp, synthetic construct
  misc_feature 1..27: note = Description of Artificial Sequence: Synthetic oligonucleotide
  source 1..27: mol_type = other DNA
tttggggtgatcaggcccaacaccagg

SEQ ID NO: 388 - DNA, 37 bp, synthetic construct
  misc_feature 1..37: note = Description of Artificial Sequence: Synthetic oligonucleotide
  source 1..37: mol_type = other DNA
cccgtcccaggaggatggcctggctgatgaggccgca

SEQ ID NO: 389 - DNA, 30 bp, synthetic construct
  misc_feature 1..30: note = Description of Artificial Sequence: Synthetic oligonucleotide
  source 1..30: mol_type = other DNA
cccgtcccaggaggatggcctgaggccgca

SEQ ID NO: 390 - DNA, 28 bp, synthetic construct
  misc_feature 1..28: note = Description of Artificial Sequence: Synthetic oligonucleotide
  source 1..28: mol_type = other DNA
cccgtcccaggaggatggcctggccgca

SEQ ID NO: 391 - DNA, 34 bp, synthetic construct
  misc_feature 1..34: note = Description of Artificial Sequence: Synthetic oligonucleotide
  source 1..34: mol_type = other DNA
cccgtcccaggaggatggcctggctgaggccgca

SEQ ID NO: 392 - DNA, 31 bp, synthetic construct
  misc_feature 1..31: note = Description of Artificial Sequence: Synthetic oligonucleotide
  source 1..31: mol_type = other DNA
cccgtcccaggaggatggcctggaggccgca

SEQ ID NO: 393 - DNA, 31 bp, synthetic construct
  misc_feature 1..31: note = Description of Artificial Sequence: Synthetic oligonucleotide
  source 1..31: mol_type = other DNA
cccgtcccaggaggatggccttgaggccgca

SEQ ID NO: 394 - DNA, 27 bp, synthetic construct
  misc_feature 1..27: note = Description of Artificial Sequence: Synthetic oligonucleotide
  source 1..27: mol_type = other DNA
cccgtcccaggaggatggcctgccgca

SEQ ID NO: 395 - DNA, 61 bp, synthetic construct
  misc_feature 1..61: note = Description of Artificial Sequence: Synthetic oligonucleotide
  source 1..61: mol_type = other DNA
gtgtggttccagaaccggaggacaaagtacaaacggcagaagctggaggaggaagggcctg

SEQ ID NO: 396 - protein, 15 aa, Butyrivibrio proteoclasticus
ARLRWWNGEENFAND

SEQ ID NO: 397 - protein, 7 aa, Butyrivibrio proteoclasticus
FLPKALF

SEQ ID NO: 398 - protein, 15 aa, unidentified
  REGION 1..15: note = Description of Unknown: Lachnospiraceae bacterium sequence
LRPNWWSPGEKFNKF

SEQ ID NO: 399 - protein, 7 aa, unidentified
  REGION 1..7: note = Description of Unknown: Lachnospiraceae bacterium sequence
FLPKLVF

SEQ ID NO: 400 - protein, 15 aa, unidentified
  REGION 1..15: note = Description of Unknown: Candidatus Falkowbacteria bacterium sequence
DLLEGWDMNKEPEYW

SEQ ID NO: 401 - protein, 6 aa, unidentified
  REGION 1..6: note = Description of Unknown: Candidatus Falkowbacteria bacterium sequence
FEGIAF

SEQ ID NO: 402 - protein, 15 aa, unidentified
  REGION 1..15: note = Description of Unknown: Candidatus Peregrinibacteria bacterium sequence
SLAGGWDVNKECSNF

SEQ ID NO: 403 - protein, 7 aa, unidentified
  REGION 1..7: note = Description of Unknown: Candidatus Peregrinibacteria bacterium sequence
MIPKCST

SEQ ID NO: 404 - protein, 15 aa, unidentified
  REGION 1..15: note = Description of Unknown: Candidatus Dojkabacteria bacterium sequence
NLLGGWSDGQERNKA

SEQ ID NO: 405 - protein, 7 aa, unidentified
  REGION 1..7: note = Description of Unknown: Candidatus Dojkabacteria bacterium sequence
KWERLIL

SEQ ID NO: 406 - protein, 15 aa, unidentified
  REGION 1..15: note = Description of Unknown: uncultured bacterium (gcode 4) sequence
QFLTWWDKDKENERL

SEQ ID NO: 407 - protein, 7 aa, unidentified
  REGION 1..7: note = Description of Unknown: uncultured bacterium (gcode 4) sequence
QLPRLLF

SEQ ID NO: 408 - protein, 15 aa, unidentified
  REGION 1..15: note = Description of Unknown: Candidatus Roizmanbacteria bacterium sequence
TLANGWDKNKESDNS

SEQ ID NO: 409 - protein, 7 aa, unidentified
  REGION 1..7: note = Description of Unknown: Candidatus Roizmanbacteria bacterium sequence
MFPKVCF

SEQ ID NO: 410 - protein, 15 aa, unidentified
  REGION 1..15: note = Description of Unknown: Parcubacteria group bacterium sequence
ALLKGWDENKEYDFM

SEQ ID NO: 411 - protein, 7 aa, unidentified
  REGION 1..7: note = Description of Unknown: Parcubacteria group bacterium sequence
DVPRLLL

SEQ ID NO: 412 - protein, 15 aa, Helcococcus kunzii
TLADGWSESKISDNR

SEQ ID NO: 413 - protein, 7 aa, Helcococcus kunzii
SIPNYPF

SEQ ID NO: 414 - protein, 15 aa, Proteocatella sphenisci
TLAKGWDANKEIDNS

SEQ ID NO: 415 - protein, 7 aa, Proteocatella sphenisci
MLPKQFL

SEQ ID NO: 416 - protein, 15 aa, unidentified
  REGION 1..15: note = Description of Unknown: Candidatus Methanomethylophilus alvus sequence
TLADGWDLNKERDNK

SEQ ID NO: 417 - protein, 7 aa, unidentified
  REGION 1..7: note = Description of Unknown: Candidatus Methanomethylophilus alvus sequence
MLPKIFV

SEQ ID NO: 418 - protein, 15 aa, Lachnospira pectinoschiza
TLASGWSRSKEFDNN

SEQ ID NO: 419 - protein, 7 aa, Lachnospira pectinoschiza
MLPKVFI

SEQ ID NO: 420 - protein, 15 aa, Eubacterium rectale
TLADGWSKSKEYSNN

SEQ ID NO: 421 - protein, 7 aa, Eubacterium rectale
MIPKVFL

SEQ ID NO: 422 - protein, 15 aa, Eubacterium eligens
TLANGWSQSKEFDNN

SEQ ID NO: 423 - protein, 7 aa, Eubacterium eligens
MLPKVFL

SEQ ID NO: 424 - protein, 15 aa, unidentified
  REGION 1..15: note = Description of Unknown: Candidatus Methanoplasma termitum sequence
TLANGWDQNKVYDYA

SEQ ID NO: 425 - protein, 7 aa, unidentified
  REGION 1..7: note = Description of Unknown: Candidatus Methanoplasma termitum sequence
NLPRVFL

SEQ ID NO: 426 - protein, 15 aa, Synergistes jonesii
ALAKGWDKNKEQNNT

SEQ ID NO: 427 - protein, 7 aa, Synergistes jonesii
ELPKVFL

SEQ ID NO: 428 - protein, 15 aa, Acidaminococcus sp.
TLASGWDVNKEKNNG

SEQ ID NO: 429 - protein, 7 aa, Acidaminococcus sp.
MIPKCST

SEQ ID NO: 430 - protein, 15 aa, Succinivibrio dextrinosolvens
QLGEGFSKSKENDCL

SEQ ID NO: 431 - protein, 7 aa, Succinivibrio dextrinosolvens
FIPKCSI

SEQ ID NO: 432 - protein, 15 aa, Porphyromonas macacae
SLLSGWDKNKELNNL

SEQ ID NO: 433 - protein, 7 aa, Porphyromonas macacae
MLPKVFF

SEQ ID NO: 434 - protein, 15 aa, Prevotella disiens
KLMTGWKSDNGTQYG

SEQ ID NO: 435 - protein, 7 aa, Prevotella disiens
RLNKVII

SEQ ID NO: 436 - protein, 15 aa, Anaerovibrio sp.
TMLAGWDYNNETANG

SEQ ID NO: 437 - protein, 7 aa, Anaerovibrio sp.
MLPKVVF

SEQ ID NO: 438 - protein, 15 aa, Moraxella bovoculi
TLLNGWDLNKEKDNF

SEQ ID NO: 439 - protein, 7 aa, Moraxella bovoculi
QFPKVFF

SEQ ID NO: 440 - protein, 15 aa, Francisella tularensis
TLANGWDKNKEPDNT

SEQ ID NO: 441 - protein, 7 aa, Francisella tularensis
MLPKVFF

SEQ ID NO: 442 - protein, 15 aa, Thiomicrospira sp.
TLLSGWDANKETANA

SEQ ID NO: 443 - protein, 7 aa, Thiomicrospira sp.
MLPKVFF

SEQ ID NO: 444 - protein, 15 aa, unidentified
  REGION 1..15: note = Description of Unknown: Lachnospiraceae bacterium sequence
QFMGGWDKDKETDYR

SEQ ID NO: 445 - protein, 7 aa, unidentified
  REGION 1..7: note = Description of Unknown: Lachnospiraceae bacterium sequence
MLPKVFF

SEQ ID NO: 446 - protein, 15 aa, unidentified
  REGION 1..15: note = Description of Unknown: Lachnospiraceae bacterium sequence
QLLGGWDVNKERDCY

SEQ ID NO: 447 - protein, 7 aa, unidentified
  REGION 1..7: note = Description of Unknown: Lachnospiraceae bacterium sequence
MFPKVFF

SEQ ID NO: 448 - protein, 15 aa, Butyrivibrio fibrisolvens
TFLDGWDYGNEEAYL

SEQ ID NO: 449 - protein, 7 aa, Butyrivibrio fibrisolvens
SIQNLMV

SEQ ID NO: 450 - protein, 15 aa, Pseudobutyrivibrio ruminis
TLLNGWDKNKETDNL

SEQ ID NO: 451 - protein, 7 aa, Pseudobutyrivibrio ruminis
MLPKVFF

SEQ ID NO: 452 - protein, 15 aa, Oribacterium sp.
TFLDGWDKNKEEANL

SEQ ID NO: 453 - protein, 7 aa, Oribacterium sp.
MLPKVFF

SEQ ID NO: 454 - protein, 15 aa, Butyrivibrio sp.
TLLNGWDKNKETDNL

SEQ ID NO: 455 - protein, 7 aa, Butyrivibrio sp.
MLPKVFF

SEQ ID NO: 456 - protein, 15 aa, unidentified
  REGION 1..15: note = Description of Unknown: Lachnospiraceae bacterium sequence
TLLNGWDRNKETDNL

SEQ ID NO: 457 - protein, 7 aa, unidentified
  REGION 1..7: note = Description of Unknown: Lachnospiraceae bacterium sequence
MLPKVFF

SEQ ID NO: 458 - protein, 15 aa, unidentified
  REGION 1..15: note = Description of Unknown: Lachnospiraceae bacterium sequence
TLLCGWSQSKEKEYM

SEQ ID NO: 459 - protein, 7 aa, unidentified
  REGION 1..7: note = Description of Unknown: Lachnospiraceae bacterium sequence
MLPKVFF

SEQ ID NO: 460 - protein, 15 aa, Leptospira inadai
TLLKGWDENREVANL

SEQ ID NO: 461 - protein, 7 aa, Leptospira inadai
QLPRIIF

SEQ ID NO: 462 - protein, 15 aa, unidentified
  REGION 1..15: note = Description of Unknown: Lachnospiraceae bacterium sequence
TLLDGWDKNKEKDNL

SEQ ID NO: 463 - protein, 7 aa, unidentified
  REGION 1..7: note = Description of Unknown: Lachnospiraceae bacterium sequence
NLPRIFL

SEQ ID NO: 464 - protein, 15 aa, Smithella sp.
TLLGGWDLNKETDNT

SEQ ID NO: 465 - protein, 7 aa, Smithella sp.
MLPKVFF

SEQ ID NO: 466 - protein, 15 aa, Flavobacterium branchiophilum
QLLNGWDANKEGDYL

SEQ ID NO: 467 - protein, 7 aa, Flavobacterium branchiophilum
MLPKVFF

SEQ ID NO: 468 - protein, 15 aa, Flavobacterium sp.
QLLNGWDANKEKDYL

SEQ ID NO: 469 - protein, 7 aa, Flavobacterium sp.
MLPKVFF

SEQ ID NO: 470 - protein, 15 aa, unidentified
  REGION 1..15: note = Description of Unknown: Bacteroidales bacterium sequence
SLLAGWDRNKEKDNL

SEQ ID NO: 471 - protein, 7 aa, unidentified
  REGION 1..7: note = Description of Unknown: Bacteroidales bacterium sequence
MLPKVYI

SEQ ID NO: 472 - protein, 15 aa, Porphyromonas crevioricanis
QLLSGWDRNKEKDNS

SEQ ID NO: 473 - protein, 7 aa, Porphyromonas crevioricanis
MLPKVFL

SEQ ID NO: 474 - protein, 15 aa, Prevotella brevis
QLLDGWDENKESTNA

SEQ ID NO: 475 - protein, 7 aa, Prevotella brevis
MVPKCTT

SEQ ID NO: 476 - protein, 15 aa, unidentified
  REGION 1..15: note = Description of Unknown: Bacteroidetes oral taxon 274 sequence
TLMDGWDLNKEPDNT

SEQ ID NO: 477 - protein, 7 aa, unidentified
  REGION 1..7: note = Description of Unknown: Bacteroidetes oral taxon 274 sequence
MLPKVFF

SEQ ID NO: 478 - protein, 15 aa, Prevotella bryantii
TLLGGWDLNKEHDNT

SEQ ID NO: 479 - protein, 7 aa, Prevotella bryantii
MLPKVFF

SEQ ID NO: 480 - protein, 15 aa, Prevotella albensis
QLLGGWDVNKEHDCA

SEQ ID NO: 481 - protein, 7 aa, Prevotella albensis
MLPKVFF

SEQ ID NO: 482 - protein, 12 aa, synthetic construct
  REGION 1..12: note = Description of Artificial Sequence: Synthetic peptide
GGGSGGGSGGGS